European Patent Application EP 4 603 505 A1, published August 20, 2025. Title: METHOD FOR MODIFYING CAPSID PROTEIN CODING GENE OF ADENO-ASSOCIATED VIRUS. Applicant: KANGLIN BIOTECH(HANGZHOU) CO., LTD. The sequence listing filed with the application follows.

SEQUENCE LISTING (26 sequences)

SEQ ID NO: 1 - DNA, 1866 bp, Adeno-associated virus 2
  source 1..1866: mol_type = genomic DNA
ctggcggggttttacgagattgtgattaaggtccccagcgaccttgacgagcatctgcccggcatttctgacagctttgtgaactgggtggccgagaaggagtgggagttgccgccagattctgacttggatctgaatctgattgagcaggcacccctgaccgtggccgagaagctgcagcgcgactttctgacggagtggcgccgtgtgagtaaggccccggaggcccttttctttgtgcaatttgagaagggagagagctacttccacttacacgtgctcgtggaaaccaccggggtgaaatccttagttttgggacgtttcctgagtcagattcgcgaaaaactgattcagagaatttaccgcgggatcgagccgactttgccaaactggttcgcggtcacaaagaccagaaacggcgccggaggcgggaacaaggtggtggacgagtgctacatccccaattacttgctccccaaaacccagcctgagctccagtgggcgtggactaatttagaacagtatttaagcgcctgtttgaatctcacggagcgtaaacggttggtggcgcagcatctgacgcacgtgtcgcagacgcaggagcagaacaaagagaatcagaatcccaattctgacgcgccggtgatcagatcaaaaacttcagccaggtacatggagctggtcgggtggctcgtggacaaggggattacctcggagaagcagtggatacaggaggaccaggcctcatacatctccttcaatgcggcctccaactcgcggtcccaaatcaaggctgccttggacaatgcgggaaagattatgagcctgactaaaaccgcccccgactacctggtgggccagcagcccgtggaggacatttccagcaatcggatttataaaattttggaactaaacgggtacgatccccaatatgcggcttccgtctttctgggatgggccacgaaaaagttcggcaagaggaacaccatctggctgtttgggcctgcaactaccgggaagaccaacatcgcggaggccatagcccacactgtgcccttctacgggtgcgtaaactggaccaatgagaactttcccttcaacgactgtgtggacaagatggtgatctggtgggaggaggggaagatgaccgccaaggtcgtggagtcggccaaagccattctcggaggaagcaaggtgcgcgtggaccagaaatgcaagtcctcggcccagatagacccgactcccgtgatcgtcacctccaacaccaacatgtgcgccgtgattgacgggaactcaacgaccttcgaacaccagcagccgttgcaagaccggatgttcaaatttgaactcacccgccgtctggatcatgactttgggaaggtcaccaagcaggaagtcaaagactttttccggtgggcaaaggatcacgtggttgaggtggagcatgaattctacgtcaaaaagggtggagccaagaaaagacccgcccccagtgacgcagatataagtgagcccaaacgggtgcgcgagtcagttgcgcagccatcgacgtcagacgcggaagcatcgatcaactacgcagacaggtaccaaaacaaatgttctcgtcacgtgggcatgaatctgatgctgtttccctgcagacaatgcgagagaatgaatcagaattcaaatatctgcttcactcacggacagaaagactgtttagagtgctttcccgtgtcagaatctcaacccgtttctgtcgtcaaaaaggcgtatcagaaactgtgctacattcatcatatcatgggaaaggtgccagacgcttgcactgcctgcgatctggtcaatgtggatttggatgactgcatctttgaacaataa

SEQ ID NO: 2 - DNA, 2217 bp, Adeno-associated virus 8
  source 1..2217: mol_type = genomic DNA
atggctgccgatggttatcttccagattggctcgaggacaacctctctgagggcattcgcgagtggtgggcgctgaaacctggagccccgaagcccaaagccaaccagcaaaagcaggacgacggccggggtctggtgcttcctggctacaagtacctcggacccttcaacggactcgacaagggggagcccgtcaacgcggcggacgcagcggccctcgagcacgacaaggcctacgaccagcagctgcaggcgggtgacaatccgtacctgcggtataaccacgccgacgccgagtttcaggagcgtctgcaagaagatacgtcttttgggggcaacctcgggcgagcagtcttccaggccaagaagcgggttctcgaacctctcggtctggttgaggaaggcgctaagacggctcctggaaagaagagaccggtagagccatcaccccagcgttctccagactcctctacgggcatcggcaagaaaggccaacagcccgccagaaaaagactcaattttggtcagactggcgactcagagtcagttccagaccctcaacctctcggagaacctccagcagcgccctctggtgtgggacctaatacaatggctgcaggcggtggcgcaccaatggcagacaataacgaaggcgccgacggagtgggtagttcctcgggaaattggcattgcgattccacatggctgggcgacagagtcatcaccaccagcacccgaacctgggccctgcccacctacaacaaccacctctacaagcaaatctccaacgggacatcgggaggagccaccaacgacaacacctacttcggctacagcaccccctgggggtattttgactttaacagattccactgccacttttcaccacgtgactggcagcgactcatcaacaacaactggggattccggcccaagagactcagcttcaagctcttcaacatccaggtcaaggaggtcacgcagaatgaaggcaccaagaccatcgccaataacctcaccagcaccatccaggtgtttacggactcggagtaccagctgccgtacgttctcggctctgcccaccagggctgcctgcctccgttcccggcggacgtgttcatgattccccagtacggctacctaacactcaacaacggtagtcaggccgtgggacgctcctccttctactgcctggaatactttccttcgcagatgctgagaaccggcaacaacttccagtttacttacaccttcgaggacgtgcctttccacagcagctacgcccacagccagagcttggaccggctgatgaatcctctgattgaccagtacctgtactacttgtctcggactcaaacaacaggaggcacggcaaatacgcagactctgggcttcagccaaggtgggcctaatacaatggccaatcaggcaaagaactggctgccaggaccctgttaccgccaacaacgcgtctcaacgacaaccgggcaaaacaacaatagcaactttgcctggactgctgggaccaaataccatctgaatggaagaaattcattggctaatcctggcatcgctatggcaacacacaaagacgacgaggagcgtttttttcccagtaacgggatcctgatttttggcaaacaaaatgctgccagagacaatgcggattacagcgatgtcatgctcaccagcgaggaagaaatcaaaaccactaaccctgtggctacagaggaatacggtatcgtggcagataacttgcagcagcaaaacacggctcctcaaattggaactgtcaacagccagggggccttacccggtatggtctggcagaaccgggacgtgtacctgcagggtcccatctgggccaagattcctcacacggacggcaacttccacccgtctccgctgatgggcggctttggcctgaaacatcctccgcctcagatcctgatcaagaacacgcctgtacctgcggatcctccgaccaccttcaaccagtcaaagctgaactctttcatcacgcaatacagcaccggacaggtcagcgtggaaattgaatgggagctgcagaaggaaaacagcaagcgctggaaccccgagatccagtacacctccaactactacaaatctacaagtgtggactttgctgttaatacagaaggcgtgtactctgaaccccgccccattggcacccgttacctcacccgtaatctgtaa

SEQ ID NO: 3 - DNA, 2217 bp, synthetic construct
  source 1..2217: mol_type = other DNA
acggctgccgacggttatctacccgactggctcgaggacaacctctctgagggcattcgcgagtggtgggcgctcaaacctggagccccgaagcccaaagccaaccagcaaaagcaggacgacggccggggtctcgtccttcctggctacaagtacctcggacccttcaacggactcgacaagggggagcccgtcaacgcggcggacgcagcggccctcgagcacgacaaggcctacgaccagcagctccaggcgggtgacaatccgtacctccggtataaccacgccgacgccgagtttcaggagcgtctccaagaggacacctcttttgggggcaacctcgggcgagcagtcttccaggccaagaagcgggttctcgagcctctcggtctcgttgaggagggcgctaagacggctcctggaaagaagagaccggtagagccatcaccccagcgttctccagactcctctacgggcatcggcaagaaaggccaacagcccgccagaaaaagactcaattttggtcagactggcgactcagagtcagttccagaccctcaacctctcggagaacctccagcagcgccctctggtgtgggacctaatacaatggctgcaggcggtggcgcaccaatggcagacaataacgaaggcgccgacggagtgggtagttcctcgggaaattggcattgcgattccacatggctgggcgacagagtcatcaccaccagcacccgaacctgggccctgcccacctacaacaaccacctctacaagcaaatctccaacgggacatcgggaggagccaccaacgacaacacctacttcggctacagcaccccctgggggtattttgactttaacagattccactgccacttttcaccacgtgactggcagcgactcatcaacaacaactggggattccggcccaagagactcagcttcaagctcttcaacatccaggtcaaggaggtcacgcagaatgaaggcaccaagaccatcgccaataacctcaccagcaccatccaggtgtttacggactcggagtaccagctgccgtacgttctcggctctgcccaccagggctgcctgcctccgttcccggcggacgtgttcatgattccccagtacggctacctaacactcaacaacggtagtcaggccgtgggacgctcctccttctactgcctggaatactttccttcgcagatgctgagaaccggcaacaacttccagtttacttacaccttcgaggacgtgcctttccacagcagctacgcccacagccagagcttggaccggctgatgaatcctctgattgaccagtacctgtactacttgtctcggactcaaacaacaggaggcacggcaaatacgcagactctgggcttcagccaaggtgggcctaatacaatggccaatcaggcaaagaactggctgccaggaccctgttaccgccaacaacgcgtctcaacgacaaccgggcaaaacaacaatagcaactttgcctggactgctgggaccaaataccatctgaatggaagaaattcattggctaatcctggcatcgctatggcaacacacaaagacgacgaggagcgtttttttcccagtaacgggatcctgatttttggcaaacaaaatgctgccagagacaatgcggattacagcgatgtcatgctcaccagcgaggaagaaatcaaaaccactaaccctgtggctacagaggaatacggtatcgtggcagataacttgcagcagcaaaacacggctcctcaaattggaactgtcaacagccagggggccttacccggtatggtctggcagaaccgggacgtgtacctgcagggtcccatctgggccaagattcctcacacggacggcaacttccacccgtctccgctgatgggcggctttggcctgaaacatcctccgcctcagatcctgatcaagaacacgcctgtacctgcggatcctccgaccaccttcaaccagtcaaagctgaactctttcatcacgcaatacagcaccggacaggtcagcgtggaaattgaatgggagctgcagaaggaaaacagcaagcgctggaaccccgagatccagtacacctccaactactacaaatctacaagtgtggactttgctgttaatacagaaggcgtgtactctgaaccccgccccattggcacccgttacctcacccgtaatctgtaa

SEQ ID NO: 4 - DNA, 2211 bp, Adeno-associated virus 6.2FF
  source 1..2211: mol_type = genomic DNA
atggctgccgatggttatcttccagattggctcgaggacaacctctctgagggcattcgcgagtggtgggacttgaaacctggagccccgaaacccaaagccaaccagcaaaagcaggacgacggccggggtctggtgcttcctggctacaagtacctcggacccttcaacggactcgacaagggggagcccgtcaacgcggcggatgcagcggccctcgagcacgacaaggcctacgaccagcagctcaaagcgggtgacaatccgtacctgcggtataaccacgccgacgccgagtttcaggagcgtctgcaagaagatacgtcttttgggggcaacctcgggcgagcagtcttccaggccaagaagagggttctcgaacctcttggtctggttgaggaaggtgctaagacggctcctggaaagaaacgtccggtagagcagtcgccacaagagccagactcctcctcgggcattggcaagacaggccagcagcccgctaaaaagagactcaattttggtcagactggcgactcagagtcagtccccgacccacaacctctcggagaacctccagcaacccccgctgctgtgggacctactacaatggcttcaggcggtggcgcaccaatggcagacaataacgaaggcgccgacggagtgggtaatgcctcaggaaattggcattgcgattccacatggctgggcgacagagtcatcaccaccagcacccgaacatgggccttgcccacctataacaaccacctctacaagcaaatctccagtgcttcaacgggggccagcaacgacaaccactacttcggctacagcaccccctgggggtattttgatttcaacagattccactgccatttctcaccacgtgactggcagcgactcatcaacaacaattggggattccggcccaagagactcaacttcaagctcttcaacatccaagtcaaggaggtcacgacgaatgatggcgtcacgaccatcgctaataaccttaccagcacggttcaagtcttctcggactcggagtaccagttgccgtacgtcctcggctctgcgcaccagggctgcctccctccgttcccggcggacgtgttcatgattccgcagtacggctacctaacgctcaacaatggcagccaggcagtgggacggtcatccttttactgcctggaatatttcccatcgcagatgctgagaacgggcaataactttaccttcagctacaccttcgaggacgtgcctttccacagcagctacgcgcacagccagagcctggaccggctgatgaatcctctcatcgaccagtacctgtatttcctgaacagaactcagaatcagtccggaagtgcccaaaacaaggacttgctgtttagccgggggtctccagctggcatgtctgttcagcccaaaaactggctacctggaccctgttaccggcagcagcgcgtttctaaaacaaaaacagacaacaacaacagcaactttacctggactggtgcttcaaaatataaccttaatgggcgtgaatctataatcaaccctggcactgctatggcctcacacaaagacgacaaagacaagttctttcccatgagcggtgtcatgatttttggaaaggagagcgccggagcttcaaacactgcattggacaatgtcatgatcacagacgaagaggaaatcaaagccactaaccccgtggccaccgaaagatttgggactgtggcagtcaatctccagagcagcagcacagaccctgcgaccggagatgtgcatgttatgggagccttacctggaatggtgtggcaagacagagacgtatacctgcagggtcctatttgggccaaaattcctcacacggatggacactttcacccgtctcctctcatgggcggctttggacttaagcacccgcctcctcagatcctcatcaaaaacacgcctgttcctgcgaatcctccggcagagttttcggctacaaagtttgcttcattcatcacccagtattccacaggacaagtgagcgtggagattgaatgggagctgcagaaagaaaacagcaaacgctggaatcccgaagtgcagtatacatctaactatgcaaaatctgccaacgttgatttcactgtggacaacaatggactttatactgagcctcgccccattggcacccgtttcctcacccgtcccctgtaa

SEQ ID NO: 5 - DNA, 2211 bp, synthetic construct
  source 1..2211: mol_type = other DNA
acggctgccgacggttatcttccagattggctcgaggacaacctctctgagggcatccgcgagtggtgggacctcaaacctggagccccgaaacccaaagccaaccagcaaaagcaggacgacggccggggtctcgtccttcctggctacaagtacctcggacccttcaacggactcgacaagggggagcccgtcaacgcggcggacgcagcggccctcgagcacgacaaggcctacgaccagcagctcaaagcgggtgacaatccgtacctccggtataaccacgccgacgccgagtttcaggagcgtctccaagaagatacctcttttgggggcaacctcgggcgagcagtcttccaggccaagaagagggttctcgaacctcttggtctcgttgaggaaggtgctaagacggctcctggaaagaaacgtccggtagagcagtcgccacaagagccagactcctcctcgggcattggcaagacaggccagcagcccgctaaaaagagactcaattttggtcagactggcgactcagagtcagtccccgacccacaacctctcggagaacctccagcaacccccgctgctgtgggacctactacaatggcttcaggcggtggcgcaccaatggcagacaataacgaaggcgccgacggagtgggtaatgcctcaggaaattggcattgcgattccacatggctgggcgacagagtcatcaccaccagcacccgaacatgggccttgcccacctataacaaccacctctacaagcaaatctccagtgcttcaacgggggccagcaacgacaaccactacttcggctacagcaccccctgggggtattttgatttcaacagattccactgccatttctcaccacgtgactggcagcgactcatcaacaacaattggggattccggcccaagagactcaacttcaagctcttcaacatccaagtcaaggaggtcacgacgaatgatggcgtcacgaccatcgctaataaccttaccagcacggttcaagtcttctcggactcggagtaccagttgccgtacgtcctcggctctgcgcaccagggctgcctccctccgttcccggcggacgtgttcatgattccgcagtacggctacctaacgctcaacaatggcagccaggcagtgggacggtcatccttttactgcctggaatatttcccatcgcagatgctgagaacgggcaataactttaccttcagctacaccttcgaggacgtgcctttccacagcagctacgcgcacagccagagcctggaccggctgatgaatcctctcatcgaccagtacctgtatttcctgaacagaactcagaatcagtccggaagtgcccaaaacaaggacttgctgtttagccgggggtctccagctggcatgtctgttcagcccaaaaactggctacctggaccctgttaccggcagcagcgcgtttctaaaacaaaaacagacaacaacaacagcaactttacctggactggtgcttcaaaatataaccttaatgggcgtgaatctataatcaaccctggcactgctatggcctcacacaaagacgacaaagacaagttctttcccatgagcggtgtcatgatttttggaaaggagagcgccggagcttcaaacactgcattggacaatgtcatgatcacagacgaagaggaaatcaaagccactaaccccgtggccaccgaaagatttgggactgtggcagtcaatctccagagcagcagcacagaccctgcgaccggagatgtgcatgttatgggagccttacctggaatggtgtggcaagacagagacgtatacctgcagggtcctatttgggccaaaattcctcacacggatggacactttcacccgtctcctctcatgggcggctttggacttaagcacccgcctcctcagatcctcatcaaaaacacgcctgttcctgcgaatcctccggcagagttttcggctacaaagtttgcttcattcatcacccagtattccacaggacaagtgagcgtggagattgaatgggagctgcagaaagaaaacagcaaacgctggaatcccgaagtgcagtatacatctaactatgcaaaatctgccaacgttgatttcactgtggacaacaatggactttatactgagcctcgccccattggcacccgtttcctcacccgtcccctgtaa

SEQ ID NO: 6 - DNA, 1388 bp, synthetic construct
  source 1..1388: mol_type = other DNA
atcgatgttgaccccaacaaaagatttataattaatcataatcacgaacaacaacaagtcaatgaaacaaataaacaagttgtcgataaaacattcataaatgacacagcaacatacaattcttgcataataaaaatttaaatgacatcatatttgagaataacaaatgacattatccctcgattgtgttttacaagtagaattctacccgtaaagcgagtttagttttgaaaaacaaatgacatcatttgtataatgacatcatcccctgattgtgttttacaagtagaattctatccgtaaagcgagttcagttttgaaaacaaatgagtcatacctaaacacgttaataatcttctgatatcagcttatgactcaagttatgagccgtgtgcaaaacatgagataagtttatgacatcatccactgatcgtgcgttacaagtagaattctactcgtaaagccagttcggttatgagccgtgtgcaaaacatgacatcagcttatgactcatacttgattgtgttttacgcgtagaattctactcgtaaagcgagttcggttatgagccgtgtgcaaaacatgacatcagcttatgagtcataattaatcgtgcgttacaagtagaattctactcgtaaagcgagttgaaggatcatatttagttgcgtttatgagataagattgaaagcacgtgtaaaatgtttcccgcgcgttggcacaactatttacaatgcggccaagttataaaagattctaatctgatatgttttaaaacacctttgcggcccgagttgtttgcgtacgtgactagcgaagaagatgtgtggaccgcagaacagatagtaaaacaaaaccctagtattggagcaataatcgatgacgtcgctgacgtagcgctttgaattccgcgcgcttcggaccgggatcgtgaccaaattccgttttgcgacgatgcagagtttttgaacaggctgctcaaacacatagatccgtacccgctcagtcggatgtattacaatgcagccaataccatgttttacacgactatggaaaactatgccgtgtccaattgcaagttcaacattgaggattacaataacatatttaaggtgatggaaaatattaggaaacacagcaacaaaaattcaaacgaccaagacgagttaaacatatatttgggagttcagtcgtcgaatgcaaagcgtaaaaaatattaataaggtaaaaattacagctacataaattacacaatttaaactgcagtctggagatacggacctttaattcaacccaacacaatatattatagttaaataagaattattatcaaatcatttgtatattaattaaaatactatactgtaaattacattttatttacaatc

SEQ ID NO: 7 - DNA, 2202 bp, synthetic construct
  source 1..2202: mol_type = other DNA
aacttgtttattgcagcttataatggttacaaataaagcaatagcatcacaaatttcacaaataaagcatttttttcactgcattctagttgtggtttgtccaaactcatcaatgtatcttatcatgtctggatctgatcactgcttgagcctaggagatccgatcatggagataattaaaatgataaccatctcgcaaataaataagtattttactgttttcgtaacagttttgtaataaaaaaacctataaatattccggattattcataccgtcccaccatcgggcgcatgatccgtacatccagccacgtcctgaacgtccaagaaaacatcatgacttccaactgtgcttccagcccctactcctgtgaggccacttcagcctgcgctgaggcccagcaactgcaggtggacacaggtggcgataagatcgtgaacaaccaggtcaccatgactcaaatcaacttcaacgcttcctacacctctgccagcactccctctcgtgctagcttcgacaactcatactcggagttctgcgacaagcaacctaacgattacttgtcttactacaaccacccaaccccggacggagctgatactgtcatctccgactctgaaaccgctgccgctagcaacttcctcgcctcagttaactcgctcactgacaacgatttggtggagtgtctgctcaagaccactgacaacctggaggaagctgtgtcctctgcctactacagcgagtcactcgaacagccagtggtcgaacaaccctctcctagctcagcttaccacgccgagtccttcgaacactctgctggtgtcaaccagccgtcggccacaggcaccaagaggaagttggacgagtacctggataactcccagggagttgtgggtcaattcaacaagatcaagttgagacctaagtacaagaagagcaccatccagtcatgcgctacactggaacaaaccatcaaccacaacactaacatctgtacagtggcttccacccaggagatcactcactacttcacaaacgacttcgccccctacctgatgaggttcgacgataacgactacaactcgaacagattctccgatcacatgtctgaaaccggttactacatgttcgtcgttaagaagtccgaggtgaagcctttcgaaatcatcttcgccaagtacgtctctaacgtggtctacgagtacacaaacaactactacatggttgacaaccgtgtgttcgttgtgaccttcgataagatccgcttcatgatcagctacaacctggttaaggagactggcatcgaaatcccacactcacaggacgtctgcaacgatgagaccgccgctcaaaactgcaagaagtgtcacttcgtggacgtccaccacacattcaaggccgctctgacctcctacttcaacctcgatatgtactacgctcagacaaccttcgtgaccttgctgcaatcactcggcgagcgtaagtgtggattcctcttgtcgaagttgtacgagatgtaccaggacaagaacctcttcactttgcccatcatgctgagccgcaaggaatcaaacgagatcgaaaccgcctctaacaacttcttcgtctcgccatacgtttcccagatcctcaagtactcggagtccgtccaattcccggacaaccctcccaacaagtacgtcgttgataacctgaacctcatcgtgaacaagaagagcactctgacatacaagtactcgtccgtcgctaacctgctcttcaacaactacaagtaccacgacaacatcgcttctaacaacaacgccgagaacctcaagaaggtcaagaaggaagacggaagcatgcacatcgttgagcagtacttgactcaaaacgtcgataacgttaagggtcacaacttcatcgtgttgtccttcaagaacgaggaaaggctgaccatcgctaagaagaacaaggagttctactggatctctggcgaaatcaaggacgttgatgtgagccaggtcatccaaaagtacaacagattcaagcaccacatgttcgtgatcggcaaggtcaaccgtcgcgagtcaactacactgcacaacaacttgctgaagctcttggccttgatcctgcagggactggtgccactctccgacgccatcacattcgccgagcaaaagctcaactgcaagtacaagaagttcgagttcaactaa

SEQ ID NO: 8 - DNA, 6792 bp, synthetic construct
  source 1..6792: mol_type = other DNA
ttctctgtcacagaatgaaaatttttctgtcatctcttcgttattaatgtttgtaattgactgaatatcaacgcttatttgcagcctgaatggcgaatgggacgcgccctgtagcggcgcattaagcgcggcgggtgtggtggttacgcgcagcgtgaccgctacacttgccagcgccctagcgcccgctcctttcgctttcttcccttcctttctcgccacgttcgccggctttccccgtcaagctctaaatcgggggctccctttagggttccgatttagtgctttacggcacctcgaccccaaaaaacttgattagggtgatggttcacgtagtgggccatcgccctgatagacggtttttcgccctttgacgttggagtccacgttctttaatagtggactcttgttccaaactggaacaacactcaaccctatctcggtctattcttttgatttataagggattttgccgatttcggcctattggttaaaaaatgagctgatttaacaaaaatttaacgcgaattttaacaaaatattaacgtttacaatttcaggtggcacttttcggggaaatgtgcgcggaacccctatttgtttatttttctaaatacattcaaatatgtatccgctcatgagacaataaccctgataaatgcttcaataatattgaaaaaggaagagtatgagtattcaacatttccgtgtcgcccttattcccttttttgcggcattttgccttcctgtttttgctcacccagaaacgctggtgaaagtaaaagatgctgaagatcagttgggtgcacgagtgggttacatcgaactggatctcaacagcggtaagatccttgagagttttcgccccgaagaacgttttccaatgatgagcacttttaaagttctgctatgtggcgcggtattatcccgtattgacgccgggcaagagcaactcggtcgccgcatacactattctcagaatgacttggttgagtactcaccagtcacagaaaagcatcttacggatggcatgacagtaagagaattatgcagtgctgccataaccatgagtgataacactgcggccaacttacttctgacaacgatcggaggaccgaaggagctaaccgcttttttgcacaacatgggggatcatgtaactcgccttgatcgttgggaaccggagctgaatgaagccataccaaacgacgagcgtgacaccacgatgcctgtagcaatggcaacaacgttgcgcaaactattaactggcgaactacttactctagcttcccggcaacaattaatagactggatggaggcggataaagttgcaggaccacttctgcgctcggcccttccggctggctggtttattgctgataaatctggagccggtgagcgtgggtctcgcggtatcattgcagcactggggccagatggtaagccctcccgtatcgtagttatctacacgacggggagtcaggcaactatggatgaacgaaatagacagatcgctgagataggtgcctcactgattaagcattggtaactgtcagaccaagtttactcatatatactttagattgatttaaaacttcatttttaatttaaaaggatctaggtgaagatcctttttgataatctcatgaccaaaatcccttaacgtgagttttcgttccactgagcgtcagaccccgtagaaaagatcaaaggatcttcttgagatcctttttttctgcgcgtaatctgctgcttgcaaacaaaaaaaccaccgctaccagcggtggtttgtttgccggatcaagagctaccaactctttttccgaaggtaactggcttcagcagagcgcagataccaaatactgtccttctagtgtagccgtagttaggccaccacttcaagaactctgtagcaccgcctacatacctcgctctgctaatcctgttaccagtggctgctgccagtggcgataagtcgtgtcttaccgggttggactcaagacgatagttaccggataaggcgcagcggtcgggctgaacggggggttcgtgcacacagcccagcttggagcgaacgacctacaccgaactgagatacctacagcgtgagcattgagaaagcgccacgcttcccgaagggagaaaggcggacaggtatccggtaagcggcagggtcggaacaggagagcgcacgagggagcttccagggggaaacgcctggtatctttatagtcctgtcgggtttcgccacctctgacttgagcgtcgatttttgtgatgctcgtcaggggggcggagcctatggaaaaacgccagcaacgcggcctttttacggttcctggccttttgctggccttttgctcacatgttctttcctgcgttatcccctgattctgtggataaccgtattaccgcctttgagtgagctgataccgctcgccgcagccgaacgaccgagcgcagcgagtcagtgagcgaggaagcggaagagcgcctgatgcggtattttctccttacgcatctgtgcggtatttcacaccgcagaccagccgcgtaacctggcaaaatcggttacggttgagtaataaatggatgccctgcgtaagcgggtgtgggcggacaataaagtcttaaactgaacaaaatagatctaaactatgacaataaagtcttaaactagacagaatagttgtaaactgaaatcagtccagttatgctgtgaaaaagcatactggacttttgttatggctaaagcaaactcttcattttctgaagtgcaaattgcccgtcgtattaaagaggggcgtggccaagggcatggtaaagactatattcgcggcgttgtgacaatttaccgaacaactccgcggccgggaagccgatctcggcttgaacgaattgttaggtggcggtacttgggtcgatatcaaagtgcatcacttcttcccgtatgcccaactttgtatagagagccactgcgggatcgtcaccgtaatctgcttgcacgtagatcacataagcaccaagcgcgttggcctcatgcttgaggagattgatgagcgcggtggcaatgccctgcctccggtgctcgccggagactgcgagatcatagatatagatctcactacgcggctgctcaaacctgggcagaacgtaagccgcgagagcgccaacaaccgcttcttggtcgaaggcagcaagcgcgatgaatgtcttactacggagcaagttcccgaggtaatcggagtccggctgatgttgggagtaggtggctacgtctccgaactcacgaccgaaaagatcaagagcagcccgcatggatttgacttggtcagggccgagcctacatgtgcgaatgatgcccatacttgagccacctaactttgttttagggcgactgccctgctgcgtaacatcgttgctgctgcgtaacatcgttgctgctccataacatcaaacatcgacccacggcgtaacgcgcttgctgcttggatgcccgaggcatagactgtacaaaaaaacagtcataacaagccatgaaaaccgccactgcgccgttaccaccgctgcgttcggtcaaggttctggaccagttgcgtgagcgcatacgctacttgcattacagtttacgaaccgaacaggcttatgtcaactgggttcgtgccttcatccgtttccacggtgtgcgtcacccggcaaccttgggcagcagcgaagtcgaggcatttctgtcctggctggcgaacgagcgcaaggtttcggtctccacgcatcgtcaggcattggcggccttgctgttcttctacggcaaggtgctgtgcacggatctgccctggcttcaggagatcggtagacctcggccgtcgcggcgcttgccggtggtgctgaccccggatgaagtggttcgcatcctcggttttctggaaggcgagcatcgtttgttcgcccaggactctagctatagttctagtggttggcctacgtacccgtagtggctatggcagggcttgccgccccgacgttggctgcgagccctgggccttcacccgaacttgggggttggggtggggaaaaggaagaaacgcgggcgtattggtcccaatggggtctcggtggggtatcgacagagtgccagccctgggaccgaaccccgcgtttatgaacaaacgacccaacacccgtgcgttttattctgtctttttattgccgtcatagcgcgggttccttccggtattgtctccttccgtgtttcagttagcctcccccatctcccggtaccccgctacagggcgcgtactatggttgctttgacgtatgcggtgtgaaataccgcacagatgcgtaaggagaaaataccgcatcaggcgcccctgcaggcagctgcgcgctcgctcgctcactgaggccgcccgggcaaagcccgggcgtcgggcgacctttggtcgcccggcctcagtgagcgagcgagcgcgcagagagggagtggccaactccatcactaggggttcctacgcgttagttattaatagtaatcaattacggggtcattagttcatagcccatatatggagttccgcgttacataacttacggtaaatggcccgcctggctgaccgcccaacgacccccgcccattgacgtcaataatgacgtatgttcccatagtaacgccaatagggactttccattgacgtcaatgggtggagtatttacggtaaactgcccacttggcagtacatcaagtgtatcatatgccaagtacgccccctattgacgtcaatgacggtaaatggcccgcctggcattatgcccagtacatgaccttatgggactttcctacttggcagtacatctacgtattagtcatcgctattaccatggtgatgcggttttggcagtacatcaatgggcgtggatagcggtttgactcacggggatttccaagtctccaccccattgacgtcaatgggagtttgttttggcaccaaaatcaacgggactttccaaaatgtcgtaacaactccgccccattgacgcaaatgggcggtaggcgtgtacggtgggaggtctatataagcagagctggtttagtgaaccgtcagatccgctagcgctaccggtcgccaccatggtgagcaagggcgaggagctgttcaccggggtggtgcccatcctggtcgagctggacggcgacgtaaacggccacaagttcagcgtgtccggcgagggcgagggcgatgccacctacggcaagctgaccctgaagttcatctgcaccaccggcaagctgcccgtgccctggcccaccctcgtgaccaccctgacctacggcgtgcagtgcttcagccgctaccccgaccacatgaagcagcacgacttcttcaagtccgccatgcccgaaggctacgtccaggagcgcaccatcttcttcaaggacgacggcaactacaagacccgcgccgaggtgaagttcgagggcgacaccctggtgaaccgcatcgagctgaagggcatcgacttcaaggaggacggcaacatcctggggcacaagctggagtacaactacaacagccacaacgtctatatcatggccgacaagcagaagaacggcatcaaggtgaacttcaagatccgccacaacatcgaggacggcagcgtgcagctcgccgaccactaccagcagaacacccccatcggcgacggccccgtgctgctgcccgacaaccactacctgagcacccagtccgccctgagcaaagaccccaacgagaagcgcgatcacatggtcctgctggagttcgtgaccgccgccgggatcactctcggcatggacgagctgtacaagtaggtcgacgtttatttgtgaaatttgtgatgctattgctttatttgtaaccatctagctttatttgtgaaatttgtgatgctattgctttatttgtaaccattataagctgcaataaacaagttaacaacaacaattgcattcattttatgtttcaggttcagggggagatgtgggaggttttttaaagtttaaacaggaacccctagtgatggagttggccactccctctctgcgcgctcgctcgctcactgaggccgggcgaccaaaggtcgcccgacgcccgggcggcctcagtgagcgagcgagcgcgcagctgcctgcaggacatgtgagcaaaaggccagcaaaaggccaggaaccgtaaaaaggccgcgttgctggcgtctagagcctgcagtctcgacaagcttgtcgagaagtactagaggatcataatcagccataccacatttgtagaggttttacttgctttaaaaaacctcccacacctccccctgaacctgaaacataaaatgaatgcaattgttgttgttaacttgtttattgcagcttataatggttacaaataaagcaatagcatcacaaatttcacaaataaagcatttttttcactgcattctagttgtggtttgtccaaactcatcaatgtatcttatcatgtctggatctgatcactgcttgagcctaggagatccgaaccagataagtgaaatctagttccaaactattttgtcatttttaattttcgtattagcttacgacgctacacccagttcccatctattttgtcactcttccctaaataatccttaaaaactccatttccacccctcccagttcccaactattttgtccgcccacagcggggcatttttcttcctgttatgtttttaatcaaacatcctgccaactccatgtgacaaaccgtcatcttcggctacttt

SEQ ID NO: 9 - DNA, 12825 bp, synthetic construct
  source 1..12825: mol_type = other DNA
ggaccagttgcgtgagcgcatacgctacttgcattacagtttacgaaccgaacaggcttatgtcaactgggttcgtgccttcatccgtttccacggtgtgcgtcacccggcaaccttgggcagcagcgaagtcgaggcatttctgtcctggctggcgaacgagcgcaaggtttcggtctccacgcatcgtcaggcattggcggccttgctgttcttctacggcaaggtgctgtgcacggatctgccctggcttcaggagatcggtagacctcggccgtcgcggcgcttgccggtggtgctgaccccggatgaagtggttcgcatcctcggttttctggaaggcgagcatcgtttgttcgcccaggactctagctatagttctagtggttggcctacgtacccgtagtggctatggcagggcttgccgccccgacgttggctgcgagccctgggccttcacccgaacttgggggttggggtggggaaaaggaagaaacgcgggcgtattggtcccaatggggtctcggtggggtatcgacagagtgccagccctgggaccgaaccccgcgtttatgaacaaacgacccaacacccgtgcgttttattctgtctttttattgccgtcatagcgcgggttccttccggtattgtctccttccgtgtttcagttagcctcccccatctcccggtaccgcatgccttagttgaactcgaacttcttgtacttgcagttgagcttttgctcggcgaatgtgatggcgtcggagagtggcaccagtccctgcaggatcaaggccaagagcttcagcaagttgttgtgcagtgtagttgactcgcgacggttgaccttgccgatcacgaacatgtggtgcttgaatctgttgtacttttggatgacctggctcacatcaacgtccttgatttcgccagagatccagtagaactccttgttcttcttagcgatggtcagcctttcctcgttcttgaaggacaacacgatgaagttgtgacccttaacgttatcgacgttttgagtcaagtactgctcaacgatgtgcatgcttccgtcttccttcttgaccttcttgaggttctcggcgttgttgttagaagcgatgttgtcgtggtacttgtagttgttgaagagcaggttagcgacggacgagtacttgtatgtcagagtgctcttcttgttcacgatgaggttcaggttatcaacgacgtacttgttgggagggttgtccgggaattggacggactccgagtacttgaggatctgggaaacgtatggcgagacgaagaagttgttagaggcggtttcgatctcgtttgattccttgcggctcagcatgatgggcaaagtgaagaggttcttgtcctggtacatctcgtacaacttcgacaagaggaatccacacttacgctcgccgagtgattgcagcaaggtcacgaaggttgtctgagcgtagtacatatcgaggttgaagtaggaggtcagagcggccttgaatgtgtggtggacgtccacgaagtgacacttcttgcagttttgagcggcggtctcatcgttgcagacgtcctgtgagtgtgggatttcgatgccagtctccttaaccaggttgtagctgatcatgaagcggatcttatcgaaggtcacaacgaacacacggttgtcaaccatgtagtagttgtttgtgtactcgtagaccacgttagagacgtacttggcgaagatgatttcgaaaggcttcacctcggacttcttaacgacgaacatgtagtaaccggtttcagacatgtgatcggagaatctgttcgagttgtagtcgttatcgtcgaacctcatcaggtagggggcgaagtcgtttgtgaagtagtgagtgatctcctgggtggaagccactgtacagatgttagtgttgtggttgatggtttgttccagtgtagcgcatgactggatggtgctcttcttgtacttaggtctcaacttgatcttgttgaattgacccacaactccctgggagttatccaggtactcgtccaacttcctcttggtgcctgtggccgacggctggttgacaccagcagagtgttcgaaggactcggcgtggtaagctgagctaggagagggttgttcgaccactggctgttcgagtgactcgctgtagtaggcagaggacacagcttcctccaggttgtcagtggtcttgagcagacactccaccaaatcgttgtcagtgagcgagttaactgaggcgaggaagttgctagcggcagcggtttcagagtcggagatgacagtatcagctccgtccggggttgggtggttgtagtaagacaagtaatcgttaggttgcttgtcgcagaactccgagtatgagttgtcgaagctagcacgagagggagtgctggcagaggtgtaggaagcgttgaagttgatttgagtcatggtgacctggttgttcacgatcttatcgccacctgtgtccacctgcagttgctgggcctcagcgcaggctgaagtggcctcacaggagtaggggctggaagcacagttggaagtcatgatgttttcttggacgttcaggacgtggctggatgtacggatcatgcgcccgatggtgggacggtatgaataatccggaatatttataggtttttttattacaaaactgttacgaaaacagtaaaatacttatttatttgcgagatggttatcattttaattatctccatgatcggatctcctaggctcaagcagtgatcagatccagacatgataagatacattgatgagtttggacaaaccacaactagaatgcagtgaaaaaaatgctttatttgtgaaatttgtgatgctattgctttatttgtaaccattataagctgcaataaacaagttaacaacaacaattgcatttgtctagtacttctcgacggtaccgcatgctatgcatcagctgctagcaccatggctcgagttacagattacgggtgaggtaacgggtgccaatggggcggggttcagagtacacgccttctgtattaacagcaaagtccacacttgtagatttgtagtagttggaggtgtactggatctcggggttccagcgcttgctgttttccttctgcagctcccattcaatttccacgctgacctgtccggtgctgtattgcgtgatgaaagagttcagctttgactggttgaaggtggtcggaggatccgcaggtacaggcgtgttcttgatcaggatctgaggcggaggatgtttcaggccaaagccgcccatcagcggagacgggtggaagttgccgtccgtgtgaggaatcttggcccagatgggaccctgcaggtacacgtcccggttctgccagaccataccgggtaaggccccctggctgttgacagttccaatttgaggagccgtgttttgctgctgcaagttatctgccacgataccgtattcctctgtagccacagggttagtggttttgatttcttcctcgctggtgagcatgacatcgctgtaatccgcattgtctctggcagcattttgtttgccaaaaatcaggatcccgttactgggaaaaaaacgctcctcgtcgtctttgtgtgttgccatagcgatgccaggattagccaatgaatttcttccattcagatggtatttggtcccagcagtccaggcaaagttgctattgttgttttgcccggttgtcgttgagacgcgttgttggcggtaacagggtcctggcagccagttctttgcctgattggccattgtattaggcccaccttggctgaagcccagagtctgcgtatttgccgtgcctcctgttgtttgagtccgagacaagtagtacaggtactggtcaatcagaggattcatcagccggtccaagctctggctgtgggcgtagctgctgtggaaaggcacgtcctcgaaggtgtaagtaaactggaagttgttgccggttctcagcatctgcgaaggaaagtattccaggcagtagaaggaggagcgtcccacggcctgactaccgttgttgagtgttaggtagccgtactggggaatcatgaacacgtccgccgggaacggaggcaggcagccctggtgggcagagccgagaacgtacggcagctggtactccgagtccgtaaacacctggatggtgctggtgaggttattggcgatggtcttggtgccttcattctgcgtgacctccttgacctggatgttgaagagcttgaagctgagtctcttgggccggaatccccagttgttgttgatgagtcgctgccagtcacgtggtgaaaagtggcagtggaatctgttaaagtcaaaatacccccagggggtgctgtagccgaagtaggtgttgtcgttggtggctcctcccgatgtcccgttggagatttgcttgtagaggtggttgttgtaggtgggcagggcccaggttcgggtgctggtggtgatgactctgtcgcccagccatgtggaatcgcaatgccaatttcccgaggaactacccactccgtcggcgccttcgttattgtctgccattggtgcgccaccgcctgcagccattgtattaggtcccacaccagagggcgctgctggaggttctccgagaggttgagggtctggaactgactctgagtcgccagtctgaccaaaattgagtctttttctggcgggctgttggcctttcttgccgatgcccgtagaggagtctggagaacgctggggtgatggctctaccggtctcttctttccaggagccgtcttagcgccttcctcaaccagaccgagaggttcgagaacccgcttcttggcctggaagactgctcgcccgaggttgcccccaaaagacgtatcttcttgcagacgctcctgaaactcggcgtcggcgtggttataccgcaggtacggattgtcacccgcctgcagctgctggtcgtaggccttgtcgtgctcgagggccgctgcgtccgccgcgttgacgggctcccccttgtcgagtccgttgaagggtccgaggtacttgtagccaggaagcaccagaccccggccgtcgtcctgcttttgctggttggctttgggcttcggggctccaggtttcagcgcccaccactcgcgaatgccctcagagaggttgtcctcgagccaatctggaagataaccatcggcagccatggcggctcaagtcttcgtcgagtgattgtaaataaaatgtaatttacagtatagtattttaattaatatacaaatgatttgataataattcttatttaactataatatattgtgttgggttgaattaaaggtccgtatctccagactgcagtttaaattgtgtaatttatgtagctgtaatttttaccttattaatattttttacgctttgcattcgacgactgaactcccaaatatatgtttaactcgtcttggtcgtttgaatttttgttgctgtgtttcctaatattttccatcaccttaaatatgttattgtaatcctcaatgttgaacttgcaattggacacggcatagttttccatagtcgtgtaaaacatggtattggctgcattgtaatacatccgactgagcgggtacggatctatgtgtttgagcagcctgttcaaaaactctgcatcgtcgcaaaacggaatttggtcacgatcccggtccgaagcgcgcggaattcaaagcgctacgtcagcgacgtcatcgattattgctccaatactagggttttgttttactatctgttctgcggtccacacatcttcttcgctagtcacgtacgcaaacaactcgggccgcaaaggtgttttaaaacatatcagattagaatcttttataacttggccgcattgtaaatagttgtgccaacgcgcgggaaacattttacacgtgctttcaatcttatctcataaacgcaactaaatatgatccttcaactcgctttacgagtagaattctacttgtaacgcacgattaattatgactcataagctgatgtcatgttttgcacacggctcataaccgaactcgctttacgagtagaattctacgcgtaaaacacaatcaagtatgagtcataagctgatgtcatgttttgcacacggctcataaccgaactggctttacgagtagaattctacttgtaacgcacgatcagtggatgatgtcataaacttatctcatgttttgcacacggctcataacttgagtcataagctgatatcagaagattattaacgtgtttaggtatgactcatttgttttcaaaactgaactcgctttacggatagaattctacttgtaaaacacaatcaggggatgatgtcattatacaaatgatgtcatttgtttttcaaaactaaactcgctttacgggtagaattctacttgtaaaacacaatcgagggataatgtcatttgttattctcaaatatgatgtcatttaaatttttattatgcaagaattgtatgttgctgtgtcatttatgaatgttttatcgacaacttgtttatttgtttcattgacttgttgttgttcgtgattatgattaattataaatcttttgttggggtcaacatcgatgtatacgccgctacagggcgcgtactatggttgctttgacgtatgcgggcggccgctctagagatcatggagataattaaaatgataaccatctcgcaaataaataagtattttactgttttcgtaacagttttgtaataaaaaaacctataaatattccggattattcataccgtcccaccatcgggcgcggatccgccgccctggcggggttttacgagattgtgattaaggtccccagcgaccttgacgagcatctgcccggcatttctgacagctttgtgaactgggtggccgagaaggagtgggagttgccgccagattctgacttggatctgaatctgattgagcaggcacccctgaccgtggccgagaagctgcagcgcgactttctgacggagtggcgccgtgtgagtaaggccccggaggcccttttctttgtgcaatttgagaagggagagagctacttccacttacacgtgctcgtggaaaccaccggggtgaaatccttagttttgggacgtttcctgagtcagattcgcgaaaaactgattcagagaatttaccgcgggatcgagccgactttgccaaactggttcgcggtcacaaagaccagaaacggcgccggaggcgggaacaaggtggtggacgagtgctacatccccaattacttgctccccaaaacccagcctgagctccagtgggcgtggactaatttagaacagtatttaagcgcctgtttgaatctcacggagcgtaaacggttggtggcgcagcatctgacgcacgtgtcgcagacgcaggagcagaacaaagagaatcagaatcccaattctgacgcgccggtgatcagatcaaaaacttcagccaggtacatggagctggtcgggtggctcgtggacaaggggattacctcggagaagcagtggatacaggaggaccaggcctcatacatctccttcaatgcggcctccaactcgcggtcccaaatcaaggctgccttggacaatgcgggaaagattatgagcctgactaaaaccgcccccgactacctggtgggccagcagcccgtggaggacatttccagcaatcggatttataaaattttggaactaaacgggtacgatccccaatatgcggcttccgtctttctgggatgggccacgaaaaagttcggcaagaggaacaccatctggctgtttgggcctgcaactaccgggaagaccaacatcgcggaggccatagcccacactgtgcccttctacgggtgcgtaaactggaccaatgagaactttcccttcaacgactgtgtggacaagatggtgatctggtgggaggaggggaagatgaccgccaaggtcgtggagtcggccaaagccattctcggaggaagcaaggtgcgcgtggaccagaaatgcaagtcctcggcccagatagacccgactcccgtgatcgtcacctccaacaccaacatgtgcgccgtgattgacgggaactcaacgaccttcgaacaccagcagccgttgcaagaccggatgttcaaatttgaactcacccgccgtctggatcatgactttgggaaggtcaccaagcaggaagtcaaagactttttccggtgggcaaaggatcacgtggttgaggtggagcatgaattctacgtcaaaaagggtggagccaagaaaagacccgcccccagtgacgcagatataagtgagcccaaacgggtgcgcgagtcagttgcgcagccatcgacgtcagacgcggaagcatcgatcaactacgcagacaggtaccaaaacaaatgttctcgtcacgtgggcatgaatctgatgctgtttccctgcagacaatgcgagagaatgaatcagaattcaaatatctgcttcactcacggacagaaagactgtttagagtgctttcccgtgtcagaatctcaacccgtttctgtcgtcaaaaaggcgtatcagaaactgtgctacattcatcatatcatgggaaaggtgccagacgcttgcactgcctgcgatctggtcaatgtggatttggatgactgcatctttgaacaataatctagagcctgcagtctcgacaagcttgtcgagaagtactagaggatcataatcagccataccacatttgtagaggttttacttgctttaaaaaacctcccacacctccccctgaacctgaaacataaaatgaatgcaattgttgttgttaacttgtttattgcagcttataatggttacaaataaagcaatagcatcacaaatttcacaaataaagcatttttttcactgcattctagttgtggtttgtccaaactcatcaatgtatcttatcatgtctggatctgatcactgcttgagcctaggagatccgaaccagataagtgaaatctagttccaaactattttgtcatttttaattttcgtattagcttacgacgctacacccagttcccatctattttgtcactcttccctaaataatccttaaaaactccatttccacccctcccagttcccaactattttgtccgcccacagcggggcatttttcttcctgttatgtttttaatcaaacatcctgccaactccatgtgacaaaccgtcatcttcggctactttttctctgtcacagaatgaaaatttttctgtcatctcttcgttattaatgtttgtaattgactgaatatcaacgcttatttgcagcctgaatggcgaatgggacgcgccctgtagcggcgcattaagcgcggcgggtgtggtggttacgcgcagcgtgaccgctacacttgccagcgccctagcgcccgctcctttcgctttcttcccttcctttctcgccacgttcgccggctttccccgtcaagctctaaatcgggggctccctttagggttccgatttagtgctttacggcacctcgaccccaaaaaacttgattagggtgatggttcacgtagtgggccatcgccctgatagacggtttttcgccctttgacgttggagtccacgttctttaatagtggactcttgttccaaactggaacaacactcaaccctatctcggtctattcttttgatttataagggattttgccgatttcggcctattggttaaaaaatgagctgatttaacaaaaatttaacgcgaattttaacaaaatattaacgtttacaatttcaggtggcacttttcggggaaatgtgcgcggaacccctatttgtttatttttctaaatacattcaaatatgtatccgctcatgagacaataaccctgataaatgcttcaataatattgaaaaaggaagagtatgagtattcaacatttccgtgtcgcccttattcccttttttgcggcattttgccttcctgtttttgctcacccagaaacgctggtgaaagtaaaagatgctgaagatcagttgggtgcacgagtgggttacatcgaactggatctcaacagcggtaagatccttgagagttttcgccccgaagaacgttttccaatgatgagcacttttaaagttctgctatgtggcgcggtattatcccgtattgacgccgggcaagagcaactcggtcgccgcatacactattctcagaatgacttggttgagtactcaccagtcacagaaaagcatcttacggatggcatgacagtaagagaattatgcagtgctgccataaccatgagtgataacactgcggccaacttacttctgacaacgatcggaggaccgaaggagctaaccgcttttttgcacaacatgggggatcatgtaactcgccttgatcgttgggaaccggagctgaatgaagccataccaaacgacgagcgtgacaccacgatgcctgtagcaatggcaacaacgttgcgcaaactattaactggcgaactacttactctagcttcccggcaacaattaatagactggatggaggcggataaagttgcaggaccacttctgcgctcggcccttccggctggctggtttattgctgataaatctggagccggtgagcgtgggtctcgcggtatcattgcagcactggggccagatggtaagccctcccgtatcgtagttatctacacgacggggagtcaggcaactatggatgaacgaaatagacagatcgctgagataggtgcctcactgattaagcattggtaactgtcagaccaagtttactcatatatactttagattgatttaaaacttcatttttaatttaaaaggatctaggtgaagatcctttttgataatctcatgaccaaaatcccttaacgtgagttttcgttccactgagcgtcagaccccgtagaaaagatcaaaggatcttcttgagatcctttttttctgcgcgtaatctgctgcttgcaaacaaaaaaaccaccgctaccagcggtggtttgtttgccggatcaagagctaccaactctttttccgaaggtaactggcttcagcagagcgcagataccaaatactgtccttctagtgtagccgtagttaggccaccacttcaagaactctgtagcaccgcctacatacctcgctctgctaatcctgttaccagtggctgctgccagtggcgataagtcgtgtcttaccgggttggactcaagacgatagttaccggataaggcgcagcggtcgggctgaacggggggttcgtgcacacagcccagcttggagcgaacgacctacaccgaactgagatacctacagcgtgagcattgagaaagcgccacgcttcccgaagggagaaaggcggacaggtatccggtaagcggcagggtcggaacaggagagcgcacgagggagcttccagggggaaacgcctggtatctttatagtcctgtcgggtttcgccacctctgacttgagcgtcgatttttgtgatgctcgtcaggggggcggagcctatggaaaaacgccagcaacgcggcctttttacggttcctggccttttgctggccttttgctcacatgttctttcctgcgttatcccctgattctgtggataaccgtattaccgcctttgagtgagctgataccgctcgccgcagccgaacgaccgagcgcagcgagtcagtgagcgaggaagcggaagagcgcctgatgcggtattttctccttacgcatctgtgcggtatttcacaccgcagaccagccgcgtaacctggcaaaatcggttacggttgagtaataaatggatgccctgcgtaagcgggtgtgggcggacaataaagtcttaaactgaacaaaatagatctaaactatgacaataaagtcttaaactagacagaatagttgtaaactgaaatcagtccagttatgctgtgaaaaagcatactggacttttgttatggctaaagcaaactcttcattttctgaagtgcaaattgcccgtcgtattaaagaggggcgtggccaagggcatggtaaagactatattcgcggcgttgtgacaatttaccgaacaactccgcggccgggaagccgatctcggcttgaacgaattgttaggtggcggtacttgggtcgatatcaaagtgcatcacttcttcccgtatgcccaactttgtatagagagccactgcgggatcgtcaccgtaatctgcttgcacgtagatcacataagcaccaagcgcgttggcctcatgcttgaggagattgatgagcgcggtggcaatgccctgcctccggtgctcgccggagactgcgagatcatagatatagatctcactacgcggctgctcaaacctgggcagaacgtaagccgcgagagcgccaacaaccgcttcttggtcgaaggcagcaagcgcgatgaatgtcttactacggagcaagttcccgaggtaatcggagtccggctgatgttgggagtaggtggctacgtctccgaactcacgaccgaaaagatcaagagcagcccgcatggatttgacttggtcagggccgagcctacatgtgcgaatgatgcccatacttgagccacctaactttgttttagggcgactgccctgctgcgtaacatcgttgctgctgcgtaacatcgttgctgctccataacatcaaacatcgacccacggcgtaacgcgcttgctgcttggatgcccgaggcatagactgtacaaaaaaacagtcataacaagccatgaaaaccgccactgcgccgttaccaccgctgcgttcggtcaaggttct

SEQ ID NO: 10 - DNA, 12825 bp, synthetic construct
  source 1..12825: mol_type = other DNA
ggaccagttgcgtgagcgcatacgctacttgcattacagtttacgaaccgaacaggcttatgtcaactgggttcgtgccttcatccgtttccacggtgtgcgtcacccggcaaccttgggcagcagcgaagtcgaggcatttctgtcctggctggcgaacgagcgcaaggtttcggtctccacgcatcgtcaggcattggcggccttgctgttcttctacggcaaggtgctgtgcacggatctgccctggcttcaggagatcggtagacctcggccgtcgcggcgcttgccggtggtgctgaccccggatgaagtggttcgcatcctcggttttctggaaggcgagcatcgtttgttcgcccaggactctagctatagttctagtggttggcctacgtacccgtagtggctatggcagggcttgccgccccgacgttggctgcgagccctgggccttcacccgaacttgggggttggggtggggaaaaggaagaaacgcgggcgtattggtcccaatggggtctcggtggggtatcgacagagtgccagccctgggaccgaaccccgcgtttatgaacaaacgacccaacacccgtgcgttttattctgtctttttattgccgtcatagcgcgggttccttccggtattgtctccttccgtgtttcagttagcctcccccatctcccggtaccgcatgccttagttgaactcgaacttcttgtacttgcagttgagcttttgctcggcgaatgtgatggcgtcggagagtggcaccagtccctgcaggatcaaggccaagagcttcagcaagttgttgtgcagtgtagttgactcgcgacggttgaccttgccgatcacgaacatgtggtgcttgaatctgttgtacttttggatgacctggctcacatcaacgtccttgatttcgccagagatccagtagaactccttgttcttcttagcgatggtcagcctttcctcgttcttgaaggacaacacgatgaagttgtgacccttaacgttatcgacgttttgagtcaagtactgctcaacgatgtgcatgcttccgtcttccttcttgaccttcttgaggttctcggcgttgttgttagaagcgatgttgtcgtggtacttgtagttgttgaagagcaggttagcgacggacgagtacttgtatgtcagagtgctcttcttgttcacgatgaggttcaggttatcaacgacgtacttgttgggagggttgtccgggaattggacggactccgagtacttgaggatctgggaaacgtatggcgagacgaagaagttgttagaggcggtttcgatctcgtttgattccttgcggctcagcatgatgggcaaagtgaagaggttcttgtcctggtacatctcgtacaacttcgacaagaggaatccacacttacgctcgccgagtgattgcagcaaggtcacgaaggttgtctgagcgtagtacatatcgaggttgaagtaggaggtcagagcggccttgaatgtgtggtggacgtccacgaagtgacacttcttgcagttttgagcggcggtctcatcgttgcagacgtcctgtgagtgtgggatttcgatgccagtctccttaaccaggttgtagctgatcatgaagcggatcttatcgaaggtcacaacgaacacacggttgtcaaccatgtagtagttgtttgtgtactcgtagaccacgttagagacgtacttggcgaagatgatttcgaaaggcttcacctcggacttcttaacgacgaacatgtagtaaccggtttcagacatgtgatcggagaatctgttcgagttgtagtcgttatcgtcgaacctcatcaggtagggggcgaagtcgtttgtgaagtagtgagtgatctcctgggtggaagccactgtacagatgttagtgttgtggttgatggtttgttccagtgtagcgcatgactggatggtgctcttcttgtacttaggtctcaacttgatcttgttgaattgacccacaactccctgggagttatccaggtactcgtccaacttcctcttggtgcctgtggccgacggctggttgacaccagcagagtgttcgaaggactcggcgtggtaagctgagctaggagagggttgttcgaccactggctgttcgagtgactcgctgtagtaggcagaggacacagcttcctccaggttgtcagtggtcttgagcagacactccaccaaatcgttgtcagtgagcgagttaactgaggcgaggaagttgctagcggcagcggtttcagagtcggagatgacagtatcagctccgtccggggttgggtggttgtagtaagacaagtaatcgttaggttgcttgtcgcagaactccgagtatgagttgtcgaagctagcacgagagggagtgctggcagaggtgtaggaagcgttgaagttgatttgagtcatggtgacctggttgttcacgatcttatcgccacctgtgtccacctgcagttgctgggcctcagcgcaggctgaagtggcctcacaggagtaggggctggaagcacagttggaagtcatgatgttttcttggacgttcaggacgtggctggatgtacggatcatgcgcccgatggtgggacggtatgaataatccggaatatttataggtttttttattacaaaactgttacgaaaacagtaaaatacttatttatttgcgagatggttatcattttaattatctccatgatcggatctcctaggctcaagcagtgatcagatccagacatgataagatacattgatgagtttggacaaaccacaactagaatgcagtgaaaaaaatgctttatttgtgaaatttgtgatgctattgctttatttgtaaccattataagctgcaataaacaagttaacaacaacaattgcatttgtctagtacttctcgacggtaccgcatgctatgcatcagctgctagcaccatggctcgagttacagattacgggtgaggtaacgggtgccaatggggcggggttcagagtacacgccttctgtattaacagcaaagtccacacttgtagatttgtagtagttggaggtgtactggatctcggggttccagcgcttgctgttttccttctgcagctcccattcaatttccacgctgacctgtccggtgctgtattgcgtgatgaaagagttcagctttgactggttgaaggtggtcggaggatccgcaggtacaggcgtgttcttgatcaggatctgaggcggaggatgtttcaggccaaagccgcccatcagcggagacgggtggaagttgccgtccgtgtgaggaatcttggcccagatgggaccctgcaggtacacgtcccggttctgccagaccataccgggtaaggccccctggctgttgacagttccaatttgaggagccgtgttttgctgctgcaagttatctgccacgataccgtattcctctgtagccacagggttagtggttttgatttcttcctcgctggtgagcatgacatcgctgtaatccgcattgtctctggcagcattttgtttgccaaaaatcaggatcccgttactgggaaaaaaacgctcctcgtcgtctttgtgtgttgccatagcgatgccaggattagccaatgaatttcttccattcagatggtatttggtcccagcagtccaggcaaagttgctattgttgttttgcccggttgtcgttgagacgcgttgttggcggtaacagggtcctggcagccagttctttgcctgattggccattgtattaggcccaccttggctgaagcccagagtctgcgtatttgccgtgcctcctgttgtttgagtccgagacaagtagtacaggtactggtcaatcagaggattcatcagccggtccaagctctggctgtgggcgtagctgctgtggaaaggcacgtcctcgaaggtgtaagtaaactggaagttgttgccggttctcagcatctgcgaaggaaagtattccaggcagtagaaggaggagcgtcccacggcctgactaccgttgttgagtgttaggtagccgtactggggaatcatgaacacgtccgccgggaacggaggcaggcagccctggtgggcagagccgagaacgtacggcagctggtactccgagtccgtaaacacctggatggtgctggtgaggttattggcgatggtcttggtgccttcattctgcgtgacctccttgacctggatgttgaagagcttgaagctgagtctcttgggccggaatccccagttgttgttgatgagtcgctgccagtcacgtggtgaaaagtggcagtggaatctgttaaagtcaaaatacccccagggggtgctgtagccgaagtaggtgttgtcgttggtggctcctcccgatgtcccgttggagatttgcttgtagaggtggttgttgtaggtgggcagggcccaggttcgggtgctggtggtgatgactctgtcgcccagccatgtggaatcgcaatgccaatttcccgaggaactacccactccgtcggcgccttcgttattgtctgccattggtgcgccaccgcctgcagccattgtattaggtcccacaccagagggcgctgctggaggttctccgagaggttgagggtctggaactgactctgagtcgccagtctgaccaaaattgagtctttttctggcgggctgttggcctttcttgccgatgcccgtagaggagtctggagaacgctggggtgatggctctaccggtctcttctttccaggagccgtcttagcgccctcctcaacgagaccgagaggctcgagaacccgcttcttggcctggaagactgctcgcccgaggttgcccccaaaagaggtgtcctcttggagacgctcctgaaactcggcgtcggcgtggttataccggaggtacggattgtcacccgcctggagctgctggtcgtaggccttgtcgtgctcgagggccgctgcgtccgccgcgttgacgggctcccccttgtcgagtccgttgaagggtccgaggtacttgtagccaggaaggacgagaccccggccgtcgtcctgcttttgctggttggctttgggcttcggggctccaggtttgagcgcccaccactcgcgaatgccctcagagaggttgtcctcgagccagtcgggtagataaccgtcggcagccgtggcggctcaagtcttcgtcgagtgattgtaaataaaatgtaatttacagtatagtattttaattaatatacaaatgatttgataataattcttatttaactataatatattgtgttgggttgaattaaaggtccgtatctccagactgcagtttaaattgtgtaatttatgtagctgtaatttttaccttattaatattttttacgctttgcattcgacgactgaactcccaaatatatgtttaactcgtcttggtcgtttgaatttttgttgctgtgtttcctaatattttccatcaccttaaatatgttattgtaatcctcaatgttgaacttgcaattggacacggcatagttttccatagtcgtgtaaaacatggtattggctgcattgtaatacatccgactgagcgggtacggatctatgtgtttgagcagcctgttcaaaaactctgcatcgtcgcaaaacggaatttggtcacgatcccggtccgaagcgcgcggaattcaaagcgctacgtcagcgacgtcatcgattattgctccaatactagggttttgttttactatctgttctgcggtccacacatcttcttcgctagtcacgtacgcaaacaactcgggccgcaaaggtgttttaaaacatatcagattagaatcttttataacttggccgcattgtaaatagttgtgccaacgcgcgggaaacattttacacgtgctttcaatcttatctcataaacgcaactaaatatgatccttcaactcgctttacgagtagaattctacttgtaacgcacgattaattatgactcataagctgatgtcatgttttgcacacggctcataaccgaactcgctttacgagtagaattctacgcgtaaaacacaatcaagtatgagtcataagctgatgtcatgttttgcacacggctcataaccgaactggctttacgagtagaattctacttgtaacgcacgatcagtggatgatgtcataaacttatctcatgttttgcacacggctcataacttgagtcataagctgatatcagaagattattaacgtgtttaggtatgactcatttgttttcaaaactgaactcgctttacggatagaattctacttgtaaaacacaatcaggggatgatgtcattatacaaatgatgtcatttgtttttcaaaactaaactcgctttacgggtagaattctacttgtaaaacacaatcgagggataatgtcatttgttattctcaaatatgatgtcatttaaatttttattatgcaagaattgtatgttgctgtgtcatttatgaatgttttatcgacaacttgtttatttgtttcattgacttgttgttgttcgtgattatgattaattataaatcttttgttggggtcaacatcgatgtatacgccgctacagggcgcgtactatggttgctttgacgtatgcgggcggccgctctagagatcatggagataattaaaatgataaccatctcgcaaataaataagtattttactgttttcgtaacagttttgtaataaaaaaacctataaatattccggattattcataccgtcccaccatcgggcgcggatccgccgccctggcggggttttacgagattgtgattaaggtccccagcgaccttgacgagcatctgcccggcatttctgacagctttgtgaactgggtggccgagaaggagtgggagttgccgccagattctgacttggatctgaatctgattgagcaggcacccctgaccgtggccgagaagctgcagcgcgactttctgacggagtggcgccgtgtgagtaaggccccggaggcccttttctttgtgcaatttgagaagggagagagctacttccacttacacgtgctcgtggaaaccaccggggtgaaatccttagttttgggacgtttcctgagtcagattcgcgaaaaactgattcagagaatttaccgcgggatcgagccgactttgccaaactggttcgcggtcacaaagaccagaaacggcgccggaggcgggaacaaggtggtggacgagtgctacatccccaattacttgctccccaaaacccagcctgagctccagtgggcgtggactaatttagaacagtatttaagcgcctgtttgaatctcacggagcgtaaacggttggtggcgcagcatctgacgcacgtgtcgcagacgcaggagcagaacaaagagaatcagaatcccaattctgacgcgccggtgatcagatcaaaaacttcagccaggtacatggagctggtcgggtggctcgtggacaaggggattacctcggagaagcagtggatacaggaggaccaggcctcatacatctccttcaatgcggcctccaactcgcggtcccaaatcaaggctgccttggacaatgcgggaaagattatgagcctgactaaaaccgcccccgactacctggtgggccagcagcccgtggaggacatttccagcaatcggatttataaaattttggaactaaacgggtacgatccccaatatgcggcttccgtctttctgggatgggccacgaaaaagttcggcaagaggaacaccatctggctgtttgggcctgcaactaccgggaagaccaacatcgcggaggccatagcccacactgtgcccttctacgggtgcgtaaactggaccaatgagaactttcccttcaacgactgtgtggacaagatggtgatctggtgggaggaggggaagatgaccgccaaggtcgtggagtcggccaaagccattctcggaggaagcaaggtgcgcgtggaccagaaatgcaagtcctcggcccagatagacccgactcccgtgatcgtcacctccaacaccaacatgtgcgccgtgattgacgggaactcaacgaccttcgaacaccagcagccgttgcaagaccggatgttcaaatttgaactcacccgccgtctggatcatgactttgggaaggtcaccaagcaggaagtcaaagactttttccggtgggcaaaggatcacgtggttgaggtggagcatgaattctacgtcaaaaagggtggagccaagaaaagacccgcccccagtgacgcagatataagtgagcccaaacgggtgcgcgagtcagttgcgcagccatcgacgtcagacgcggaagcatcgatcaactacgcagacaggtaccaaaacaaatgttctcgtcacgtgggcatgaatctgatgctgtttccctgcagacaatgcgagagaatgaatcagaattcaaatatctgcttcactcacggacagaaagactgtttagagtgctttcccgtgtcagaatctcaacccgtttctgtcgtcaaaaaggcgtatcagaaactgtgctacattcatcatatcatgggaaaggtgccagacgcttgcactgcctgcgatctggtcaatgtggatttggatgactgcatctttgaacaataatctagagcctgcagtctcgacaagcttgtcgagaagtactagaggatcataatcagccataccacatttgtagaggttttacttgctttaaaaaacctcccacacctccccctgaacctgaaacataaaatgaatgcaattgttgttgttaacttgtttattgcagcttataatggttacaaataaagcaatagcatcacaaatttcacaaataaagcatttttttcactgcattctagttgtggtttgtccaaactcatcaatgtatcttatcatgtctggatctgatcactgcttgagcctaggagatccgaaccagataagtgaaatctagttccaaactattttgtcatttttaattttcgtattagcttacgacgctacacccagttcccatctattttgtcactcttccctaaataatccttaaaaactccatttccacccctcccagttcccaactattttgtccgcccacagcggggcatttttcttcctgttatgtttttaatcaaacatcctgccaactccatgtgacaaaccgtcatcttcggctactttttctctgtcacagaatgaaaatttttctgtcatctcttcgttattaatgtttgtaattgactgaatatcaacgcttatttgcagcctgaatggcgaatgggacgcgccctgtagcggcgcattaagcgcggcgggtgtggtggttacgcgcagcgtgaccgctacacttgccagcgccctagcgcccgctcctttcgctttcttcccttcctttctcgccacgttcgccggctttccccgtcaagctctaaatcgggggctccctttagggttccgatttagtgctttacggcacctcgaccccaaaaaacttgattagggtgatggttcacgtagtgggccatcgccctgatagacggtttttcgccctttgacgttggagtccacgttctttaatagtggactcttgttccaaactggaacaacactcaaccctatctcggtctattcttttgatttataagggattttgccgatttcggcctattggttaaaaaatgagctgatttaacaaaaatttaacgcgaattttaacaaaatattaacgtttacaatttcaggtggcacttttcggggaaatgtgcgcggaacccctatttgtttatttttctaaatacattcaaatatgtatccgctcatgagacaataaccctgataaatgcttcaataatattgaaaaaggaagagtatgagtattcaacatttccgtgtcgcccttattcccttttttgcggcattttgccttcctgtttttgctcacccagaaacgctggtgaaagtaaaagatgctgaagatcagttgggtgcacgagtgggttacatcgaactggatctcaacagcggtaagatccttgagagttttcgccccgaagaacgttttccaatgatgagcacttttaaagttctgctatgtggcgcggtattatcccgtattgacgccgggcaagagcaactcggtcgccgcatacactattctcagaatgacttggttgagtactcaccagtcacagaaaagcatcttacggatggcatgacagtaagagaattatgcagtgctgccataaccatgagtgataacactgcggccaacttacttctgacaacgatcggaggaccgaaggagctaaccgcttttttgcacaacatgggggatcatgtaactcgccttgatcgttgggaaccggagctgaatgaagccataccaaacgacgagcgtgacaccacgatgcctgtagcaatggcaacaacgttgcgcaaactattaactggcgaactacttactctagcttcccggcaacaattaatagactggatggaggcggataaagttgcaggaccacttctgcgctcggcccttccggctggctggtttattgctgataaatctggagccggtgagcgtgggtctcgcggtatcattgcagcactggggccagatggtaagccctcccgtatcgtagttatctacacgacggggagtcaggcaactatggatgaacgaaatagacagatcgctgagataggtgcctcactgattaagcattggtaactgtcagaccaagtttactcatatatactttagattgatttaaaacttcatttttaatttaaaaggatctaggtgaagatcctttttgataatctcatgaccaaaatcccttaacgtgagttttcgttccactgagcgtcagaccccgtagaaaagatcaaaggatcttcttgagatcctttttttctgcgcgtaatctgctgcttgcaaacaaaaaaaccaccgctaccagcggtggtttgtttgccggatcaagagctaccaactctttttccgaaggtaactggcttcagcagagcgcagataccaaatactgtccttctagtgtagccgtagttaggccaccacttcaagaactctgtagcaccgcctacatacctcgctctgctaatcctgttaccagtggctgctgccagtggcgataagtcgtgtcttaccgggttggactcaagacgatagttaccggataaggcgcagcggtcgggctgaacggggggttcgtgcacacagcccagcttggagcgaacgacctacaccgaactgagatacctacagcgtgagcattgagaaagcgccacgcttcccgaagggagaaaggcggacaggtatccggtaagcggcagggtcggaacaggagagcgcacgagggagcttccagggggaaacgcctggtatctttatagtcctgtcgggtttcgccacctctgacttgagcgtcgatttttgtgatgctcgtcaggggggcggagcctatggaaaaacgccagcaacgcggcctttttacggttcctggccttttgctggccttttgctcacatgttctttcctgcgttatcccctgattctgtggataaccgtattaccgcctttgagtgagctgataccgctcgccgcagccgaacgaccgagcgcagcgagtcagtgagcgaggaagcggaagagcgcctgatgcggtattttctccttacgcatctgtgcggtatttcacaccgcagaccagccgcgtaacctggcaaaatcggttacggttgagtaataaatggatgccctgcgtaagcgggtgtgggcggacaataaagtcttaaactgaacaaaatagatctaaactatgacaataaagtcttaaactagacagaatagttgtaaactgaaatcagtccagttatgctgtgaaaaagcatactggacttttgttatggctaaagcaaactcttcattttctgaagtgcaaattgcccgtcgtattaaagaggggcgtggccaagggcatggtaaagactatattcgcggcgttgtgacaatttaccgaacaactccgcggccgggaagccgatctcggcttgaacgaattgttaggtggcggtacttgggtcgatatcaaagtgcatcacttcttcccgtatgcccaactttgtatagagagccactgcgggatcgtcaccgtaatctgcttgcacgtagatcacataagcaccaagcgcgttggcctcatgcttgaggagattgatgagcgcggtggcaatgccctgcctccggtgctcgccggagactgcgagatcatagatatagatctcactacgcggctgctcaaacctgggcagaacgtaagccgcgagagcgccaacaaccgcttcttggtcgaaggcagcaagcgcgatgaatgtcttactacggagcaagttcccgaggtaatcggagtccggctgatgttgggagtaggtggctacgtctccgaactcacgaccgaaaagatcaagagcagcccgcatggatttgacttggtcagggccgagcctacatgtgcgaatgatgcccatacttgagccacctaactttgttttagggcgactgccctgctgcgtaacatcgttgctgctgcgtaacatcgttgctgctccataacatcaaacatcgacccacggcgtaacgcgcttgctgcttggatgcccgaggcatagactgtacaaaaaaacagtcataacaagccatgaaaaccgccactgcgccgttaccaccgctgcgttcggtcaaggttct

SEQ ID NO: 11 - DNA, 12819 bp, synthetic construct
  source 1..12819: mol_type = other DNA
ggaccagttgcgtgagcgcatacgctacttgcattacagtttacgaaccgaacaggcttatgtcaactgggttcgtgccttcatccgtttccacggtgtgcgtcacccggcaaccttgggcagcagcgaagtcgaggcatttctgtcctggctggcgaacgagcgcaaggtttcggtctccacgcatcgtcaggcattggcggccttgctgttcttctacggcaaggtgctgtgcacggatctgccctggcttcaggagatcggtagacctcggccgtcgcggcgcttgccggtggtgctgaccccggatgaagtggttcgcatcctcggttttctggaaggcgagcatcgtttgttcgcccaggactctagctatagttctagtggttggcctacgtacccgtagtggctatggcagggcttgccgccccgacgttggctgcgagccctgggccttcacccgaacttgggggttggggtggggaaaaggaagaaacgcgggcgtattggtcccaatggggtctcggtggggtatcgacagagtgccagccctgggaccgaaccccgcgtttatgaacaaacgacccaacacccgtgcgttttattctgtctttttattgccgtcatagcgcgggttccttccggtattgtctccttccgtgtttcagttagcctcccccatctcccggtaccgcatgccttagttgaactcgaacttcttgtacttgcagttgagcttttgctcggcgaatgtgatggcgtcggagagtggcaccagtccctgcaggatcaaggccaagagcttcagcaagttgttgtgcagtgtagttgactcgcgacggttgaccttgccgatcacgaacatgtggtgcttgaatctgttgtacttttggatgacctggctcacatcaacgtccttgatttcgccagagatccagtagaactccttgttcttcttagcgatggtcagcctttcctcgttcttgaaggacaacacgatgaagttgtgacccttaacgttatcgacgttttgagtcaagtactgctcaacgatgtgcatgcttccgtcttccttcttgaccttcttgaggttctcggcgttgttgttagaagcgatgttgtcgtggtacttgtagttgttgaagagcaggttagcgacggacgagtacttgtatgtcagagtgctcttcttgttcacgatgaggttcaggttatcaacgacgtacttgttgggagggttgtccgggaattggacggactccgagtacttgaggatctgggaaacgtatggcgagacgaagaagttgttagaggcggtttcgatctcgtttgattccttgcggctcagcatgatgggcaaagtgaagaggttcttgtcctggtacatctcgtacaacttcgacaagaggaatccacacttacgctcgccgagtgattgcagcaaggtcacgaaggttgtctgagcgtagtacatatcgaggttgaagtaggaggtcagagcggccttgaatgtgtggtggacgtccacgaagtgacacttcttgcagttttgagcggcggtctcatcgttgcagacgtcctgtgagtgtgggatttcgatgccagtctccttaaccaggttgtagctgatcatgaagcggatcttatcgaaggtcacaacgaacacacggttgtcaaccatgtagtagttgtttgtgtactcgtagaccacgttagagacgtacttggcgaagatgatttcgaaaggcttcacctcggacttcttaacgacgaacatgtagtaaccggtttcagacatgtgatcggagaatctgttcgagttgtagtcgttatcgtcgaacctcatcaggtagggggcgaagtcgtttgtgaagtagtgagtgatctcctgggtggaagccactgtacagatgttagtgttgtggttgatggtttgttccagtgtagcgcatgactggatggtgctcttcttgtacttaggtctcaacttgatcttgttgaattgacccacaactccctgggagttatccaggtactcgtccaacttcctcttggtgcctgtggccgacggctggttgacaccagcagagtgttcgaaggactcggcgtggtaagctgagctaggagagggttgttcgaccactggctgttcgagtgactcgctgtagtaggcagaggacacagcttcctccaggttgtcagtggtcttgagcagacactccaccaaatcgttgtcagtgagcgagttaactgaggcgaggaagttgctagcggcagcggtttcagagtcggagatgacagtatcagctccgtccggggttgggtggttgtagtaagacaagtaatcgttaggttgcttgtcgcagaactccgagtatgagttgtcgaagctagcacgagagggagtgctggcagaggtgtaggaagcgttgaagttgatttgagtcatggtgacctggttgttcacgatcttatcgccacctgtgtccacctgcagttgctgggcctcagcgcaggctgaagtggcctcacaggagtaggggctggaagcacagttggaagtcatgatgttttcttggacgttcaggacgtggctggatgtacggatcatgcgcccgatggtgggacggtatgaataatccggaatatttataggtttttttattacaaaactgttacgaaaacagtaaaatacttatttatttgcgagatggttatcattttaattatctccatgatcggatctcctaggctcaagcagtgatcagatccagacatgataagatacattgatgagtttggacaaaccacaactagaatgcagtgaaaaaaatgctttatttgtgaaatttgtgatgctattgctttatttgtaaccattataagctgcaataaacaagttaacaacaacaattgcatttgtctagtacttctcgacggtaccgcatgctatgcatcagctgctagcaccatggctcgagttacaggggacgggtgaggaaacgggtgccaatggggcgaggctcagtataaagtccattgttgtccacagtgaaatcaacgttggcagattttgcatagttagatgtatactgcacttcgggattccagcgtttgctgttttctttctgcagctcccattcaatctccacgctcacttgtcctgtggaatactgggtgatgaatgaagcaaactttgtagccgaaaactctgccggaggattcgcaggaacaggcgtgtttttgatgaggatctgaggaggcgggtgcttaagtccaaagccgcccatgagaggagacgggtgaaagtgtccatccgtgtgaggaattttggcccaaataggaccctgcaggtatacgtctctgtcttgccacaccattccaggtaaggctcccataacatgcacatctccggtcgcagggtctgtgctgctgctctggagattgactgccacagtcccaaatctttcggtggccacggggttagtggctttgatttcctcttcgtctgtgatcatgacattgtccaatgcagtgtttgaagctccggcgctctcctttccaaaaatcatgacaccgctcatgggaaagaacttgtctttgtcgtctttgtgtgaggccatagcagtgccagggttgattatagattcacgcccattaaggttatattttgaagcaccagtccaggtaaagttgctgttgttgttgtctgtttttgttttagaaacgcgctgctgccggtaacagggtccaggtagccagtttttgggctgaacagacatgccagctggagacccccggctaaacagcaagtccttgttttgggcacttccggactgattctgagttctgttcaggaaatacaggtactggtcgatgagaggattcatcagccggtccaggctctggctgtgcgcgtagctgctgtggaaaggcacgtcctcgaaggtgtagctgaaggtaaagttattgcccgttctcagcatctgcgatgggaaatattccaggcagtaaaaggatgaccgtcccactgcctggctgccattgttgagcgttaggtagccgtactgcggaatcatgaacacgtccgccgggaacggagggaggcagccctggtgcgcagagccgaggacgtacggcaactggtactccgagtccgagaagacttgaaccgtgctggtaaggttattagcgatggtcgtgacgccatcattcgtcgtgacctccttgacttggatgttgaagagcttgaagttgagtctcttgggccggaatccccaattgttgttgatgagtcgctgccagtcacgtggtgagaaatggcagtggaatctgttgaaatcaaaatacccccagggggtgctgtagccgaagtagtggttgtcgttgctggcccccgttgaagcactggagatttgcttgtagaggtggttgttataggtgggcaaggcccatgttcgggtgctggtggtgatgactctgtcgcccagccatgtggaatcgcaatgccaatttcctgaggcattacccactccgtcggcgccttcgttattgtctgccattggtgcgccaccgcctgaagccattgtagtaggtcccacagcagcgggggttgctggaggttctccgagaggttgtgggtcggggactgactctgagtcgccagtctgaccaaaattgagtctctttttagcgggctgctggcctgtcttgccaatgcccgaggaggagtctggctcttgtggcgactgctctaccggacgtttctttccaggagccgtcttagcaccttcctcaaccagaccaagaggttcgagaaccctcttcttggcctggaagactgctcgcccgaggttgcccccaaaagacgtatcttcttgcagacgctcctgaaactcggcgtcggcgtggttataccgcaggtacggattgtcacccgctttgagctgctggtcgtaggccttgtcgtgctcgagggccgctgcatccgccgcgttgacgggctcccccttgtcgagtccgttgaagggtccgaggtacttgtagccaggaagcaccagaccccggccgtcgtcctgcttttgctggttggctttgggtttcggggctccaggtttcaagtcccaccactcgcgaatgccctcagagaggttgtcctcgagccaatctggaagataaccatcggcagccatggcggctcaagtcttcgtcgagtgattgtaaataaaatgtaatttacagtatagtattttaattaatatacaaatgatttgataataattcttatttaactataatatattgtgttgggttgaattaaaggtccgtatctccagactgcagtttaaattgtgtaatttatgtagctgtaatttttaccttattaatattttttacgctttgcattcgacgactgaactcccaaatatatgtttaactcgtcttggtcgtttgaatttttgttgctgtgtttcctaatattttccatcaccttaaatatgttattgtaatcctcaatgttgaacttgcaattggacacggcatagttttccatagtcgtgtaaaacatggtattggctgcattgtaatacatccgactgagcgggtacggatctatgtgtttgagcagcctgttcaaaaactctgcatcgtcgcaaaacggaatttggtcacgatcccggtccgaagcgcgcggaattcaaagcgctacgtcagcgacgtcatcgattattgctccaatactagggttttgttttactatctgttctgcggtccacacatcttcttcgctagtcacgtacgcaaacaactcgggccgcaaaggtgttttaaaacatatcagattagaatcttttataacttggccgcattgtaaatagttgtgccaacgcgcgggaaacattttacacgtgctttcaatcttatctcataaacgcaactaaatatgatccttcaactcgctttacgagtagaattctacttgtaacgcacgattaattatgactcataagctgatgtcatgttttgcacacggctcataaccgaactcgctttacgagtagaattctacgcgtaaaacacaatcaagtatgagtcataagctgatgtcatgttttgcacacggctcataaccgaactggctttacgagtagaattctacttgtaacgcacgatcagtggatgatgtcataaacttatctcatgttttgcacacggctcataacttgagtcataagctgatatcagaagattattaacgtgtttaggtatgactcatttgttttcaaaactgaactcgctttacggatagaattctacttgtaaaacacaatcaggggatgatgtcattatacaaatgatgtcatttgtttttcaaaactaaactcgctttacgggtagaattctacttgtaaaacacaatcgagggataatgtcatttgttattctcaaatatgatgtcatttaaatttttattatgcaagaattgtatgttgctgtgtcatttatgaatgttttatcgacaacttgtttatttgtttcattgacttgttgttgttcgtgattatgattaattataaatcttttgttggggtcaacatcgatgtatacgccgctacagggcgcgtactatggttgctttgacgtatgcgggcggccgctctagagatcatggagataattaaaatgataaccatctcgcaaataaataagtattttactgttttcgtaacagttttgtaataaaaaaacctataaatattccggattattcataccgtcccaccatcgggcgcggatccgccgccctggcggggttttacgagattgtgattaaggtccccagcgaccttgacgagcatctgcccggcatttctgacagctttgtgaactgggtggccgagaaggagtgggagttgccgccagattctgacttggatctgaatctgattgagcaggcacccctgaccgtggccgagaagctgcagcgcgactttctgacggagtggcgccgtgtgagtaaggccccggaggcccttttctttgtgcaatttgagaagggagagagctacttccacttacacgtgctcgtggaaaccaccggggtgaaatccttagttttgggacgtttcctgagtcagattcgcgaaaaactgattcagagaatttaccgcgggatcgagccgactttgccaaactggttcgcggtcacaaagaccagaaacggcgccggaggcgggaacaaggtggtggacgagtgctacatccccaattacttgctccccaaaacccagcctgagctccagtgggcgtggactaatttagaacagtatttaagcgcctgtttgaatctcacggagcgtaaacggttggtggcgcagcatctgacgcacgtgtcgcagacgcaggagcagaacaaagagaatcagaatcccaattctgacgcgccggtgatcagatcaaaaacttcagccaggtacatggagctggtcgggtggctcgtggacaaggggattacctcggagaagcagtggatacaggaggaccaggcctcatacatctccttcaatgcggcctccaactcgcggtcccaaatcaaggctgccttggacaatgcgggaaagattatgagcctgactaaaaccgcccccgactacctggtgggccagcagcccgtggaggacatttccagcaatcggatttataaaattttggaactaaacgggtacgatccccaatatgcggcttccgtctttctgggatgggccacgaaaaagttcggcaagaggaacaccatctggctgtttgggcctgcaactaccgggaagaccaacatcgcggaggccatagcccacactgtgcccttctacgggtgcgtaaactggaccaatgagaactttcccttcaacgactgtgtggacaagatggtgatctggtgggaggaggggaagatgaccgccaaggtcgtggagtcggccaaagccattctcggaggaagcaaggtgcgcgtggaccagaaatgcaagtcctcggcccagatagacccgactcccgtgatcgtcacctccaacaccaacatgtgcgccgtgattgacgggaactcaacgaccttcgaacaccagcagccgttgcaagaccggatgttcaaatttgaactcacccgccgtctggatcatgactttgggaaggtcaccaagcaggaagtcaaagactttttccggtgggcaaaggatcacgtggttgaggtggagcatgaattctacgtcaaaaagggtggagccaagaaaagacccgcccccagtgacgcagatataagtgagcccaaacgggtgcgcgagtcagttgcgcagccatcgacgtcagacgcggaagcatcgatcaactacgcagacaggtaccaaaacaaatgttctcgtcacgtgggcatgaatctgatgctgtttccctgcagacaatgcgagagaatgaatcagaattcaaatatctgcttcactcacggacagaaagactgtttagagtgctttcccgtgtcagaatctcaacccgtttctgtcgtcaaaaaggcgtatcagaaactgtgctacattcatcatatcatgggaaaggtgccagacgcttgcactgcctgcgatctggtcaatgtggatttggatgactgcatctttgaacaataatctagagcctgcagtctcgacaagcttgtcgagaagtactagaggatcataatcagccataccacatttgtagaggttttacttgctttaaaaaacctcccacacctccccctgaacctgaaacataaaatgaatgcaattgttgttgttaacttgtttattgcagcttataatggttacaaataaagcaatagcatcacaaatttcacaaataaagcatttttttcactgcattctagttgtggtttgtccaaactcatcaatgtatcttatcatgtctggatctgatcactgcttgagcctaggagatccgaaccagataagtgaaatctagttccaaactattttgtcatttttaattttcgtattagcttacgacgctacacccagttcccatctattttgtcactcttccctaaataatccttaaaaactccatttccacccctcccagttcccaactattttgtccgcccacagcggggcatttttcttcctgttatgtttttaatcaaacatcctgccaactccatgtgacaaaccgtcatcttcggctactttttctctgtcacagaatgaaaatttttctgtcatctcttcgttattaatgtttgtaattgactgaatatcaacgcttatttgcagcctgaatggcgaatgggacgcgccctgtagcggcgcattaagcgcggcgggtgtggtggttacgcgcagcgtgaccgctacacttgccagcgccctagcgcccgctcctttcgctttcttcccttcctttctcgccacgttcgccggctttccccgtcaagctctaaatcgggggctccctttagggttccgatttagtgctttacggcacctcgaccccaaaaaacttgattagggtgatggttcacgtagtgggccatcgccctgatagacggtttttcgccctttgacgttggagtccacgttctttaatagtggactcttgttccaaactggaacaacactcaaccctatctcggtctattcttttgatttataagggattttgccgatttcggcctattggttaaaaaatgagctgatttaacaaaaatttaacgcgaattttaacaaaatattaacgtttacaatttcaggtggcacttttcggggaaatgtgcgcggaacccctatttgtttatttttctaaatacattcaaatatgtatccgctcatgagacaataaccctgataaatgcttcaataatattgaaaaaggaagagtatgagtattcaacatttccgtgtcgcccttattcccttttttgcggcattttgccttcctgtttttgctcacccagaaacgctggtgaaagtaaaagatgctgaagatcagttgggtgcacgagtgggttacatcgaactggatctcaacagcggtaagatccttgagagttttcgccccgaagaacgttttccaatgatgagcacttttaaagttctgctatgtggcgcggtattatcccgtattgacgccgggcaagagcaactcggtcgccgcatacactattctcagaatgacttggttgagtactcaccagtcacagaaaagcatcttacggatggcatgacagtaagagaattatgcagtgctgccataaccatgagtgataacactgcggccaacttacttctgacaacgatcggaggaccgaaggagctaaccgcttttttgcacaacatgggggatcatgtaactcgccttgatcgttgggaaccggagctgaatgaagccataccaaacgacgagcgtgacaccacgatgcctgtagcaatggcaacaacgttgcgcaaactattaactggcgaactacttactctagcttcccggcaacaattaatagactggatggaggcggataaagttgcaggaccacttctgcgctcggcccttccggctggctggtttattgctgataaatctggagccggtgagcgtgggtctcgcggtatcattgcagcactggggccagatggtaagccctcccgtatcgtagttatctacacgacggggagtcaggcaactatggatgaacgaaatagacagatcgctgagataggtgcctcactgattaagcattggtaactgtcagaccaagtttactcatatatactttagattgatttaaaacttcatttttaatttaaaaggatctaggtgaagatcctttttgataatctcatgaccaaaatcccttaacgtgagttttcgttccactgagcgtcagaccccgtagaaaagatcaaaggatcttcttgagatcctttttttctgcgcgtaatctgctgcttgcaaacaaaaaaaccaccgctaccagcggtggtttgtttgccggatcaagagctaccaactctttttccgaaggtaactggcttcagcagagcgcagataccaaatactgtccttctagtgtagccgtagttaggccaccacttcaagaactctgtagcaccgcctacatacctcgctctgctaatcctgttaccagtggctgctgccagtggcgataagtcgtgtcttaccgggttggactcaagacgatagttaccggataaggcgcagcggtcgggctgaacggggggttcgtgcacacagcccagcttggagcgaacgacctacaccgaactgagatacctacagcgtgagcattgagaaagcgccacgcttcccgaagggagaaaggcggacaggtatccggtaagcggcagggtcggaacaggagagcgcacgagggagcttccagggggaaacgcctggtatctttatagtcctgtcgggtttcgccacctctgacttgagcgtcgatttttgtgatgctcgtcaggggggcggagcctatggaaaaacgccagcaacgcggcctttttacggttcctggccttttgctggccttttgctcacatgttctttcctgcgttatcccctgattctgtggataaccgtattaccgcctttgagtgagctgataccgctcgccgcagccgaacgaccgagcgcagcgagtcagtgagcgaggaagcggaagagcgcctgatgcggtattttctccttacgcatctgtgcggtatttcacaccgcagaccagccgcgtaacctggcaaaatcggttacggttgagtaataaatggatgccctgcgtaagcgggtgtgggcggacaataaagtcttaaactgaacaaaatagatctaaactatgacaataaagtcttaaactagacagaatagttgtaaactgaaatcagtccagttatgctgtgaaaaagcatactggacttttgttatggctaaagcaaactcttcattttctgaagtgcaaattgcccgtcgtattaaagaggggcgtggccaagggcatggtaaagactatattcgcggcgttgtgacaatttaccgaacaactccgcggccgggaagccgatctcggcttgaacgaattgttaggtggcggtacttgggtcgatatcaaagtgcatcacttcttcccgtatgcccaactttgtatagagagccactgcgggatcgtcaccgtaatctgcttgcacgtagatcacataagcaccaagcgcgttggcctcatgcttgaggagattgatgagcgcggtggcaatgccctgcctccggtgctcgccggagactgcgagatcatagatatagatctcactacgcggctgctcaaacctgggcagaacgtaagccgcgagagcgccaacaaccgcttcttggtcgaaggcagcaagcgcgatgaatgtcttactacggagcaagttcccgaggtaatcggagtccggctgatgttgggagtaggtggctacgtctccgaactcacgaccgaaaagatcaagagcagcccgcatggatttgacttggtcagggccgagcctacatgtgcgaatgatgcccatacttgagccacctaactttgttttagggcgactgccctgctgcgtaacatcgttgctgctgcgtaacatcgttgctgctccataacatcaaacatcgacccacggcgtaacgcgcttgctgcttggatgcccgaggcatagactgtacaaaaaaacagtcataacaagccatgaaaaccgccactgcgccgttaccaccgctgcgttcggtcaaggttct

SEQ ID NO: 12 - DNA, 12819 bp, synthetic construct
  source 1..12819: mol_type = other DNA
ggaccagttgcgtgagcgcatacgctacttgcattacagtttacgaaccgaacaggcttatgtcaactgggttcgtgccttcatccgtttccacggtgtgcgtcacccggcaaccttgggcagcagcgaagtcgaggcatttctgtcctggctggcgaacgagcgcaaggtttcggtctccacgcatcgtcaggcattggcggccttgctgttcttctacggcaaggtgctgtgcacggatctgccctggcttcaggagatcggtagacctcggccgtcgcggcgcttgccggtggtgctgaccccggatgaagtggttcgcatcctcggttttctggaaggcgagcatcgtttgttcgcccaggactctagctatagttctagtggttggcctacgtacccgtagtggctatggcagggcttgccgccccgacgttggctgcgagccctgggccttcacccgaacttgggggttggggtggggaaaaggaagaaacgcgggcgtattggtcccaatggggtctcggtggggtatcgacagagtgccagccctgggaccgaaccccgcgtttatgaacaaacgacccaacacccgtgcgttttattctgtctttttattgccgtcatagcgcgggttccttccggtattgtctccttccgtgtttcagttagcctcccccatctcccggtaccgcatgccttagttgaactcgaacttcttgtacttgcagttgagcttttgctcggcgaatgtgatggcgtcggagagtggcaccagtccctgcaggatcaaggccaagagcttcagcaagttgttgtgcagtgtagttgactcgcgacggttgaccttgccgatcacgaacatgtggtgcttgaatctgttgtacttttggatgacctggctcacatcaacgtccttgatttcgccagagatccagtagaactccttgttcttcttagcgatggtcagcctttcctcgttcttgaaggacaacacgatgaagttgtgacccttaacgttatcgacgttttgagtcaagtactgctcaacgatgtgcatgcttccgtcttccttcttgaccttcttgaggttctcggcgttgttgttagaagcgatgttgtcgtggtacttgtagttgttgaagagcaggttagcgacggacgagtacttgtatgtcagagtgctcttcttgttcacgatgaggttcaggttatcaacgacgtacttgttgggagggttgtccgggaattggacggactccgagtacttgaggatctgggaaacgtatggcgagacgaagaagttgttagaggcggtttcgatctcgtttgattccttgcggctcagcatgatgggcaaagtgaagaggttcttgtcctggtacatctcgtacaacttcgacaagaggaatccacacttacgctcgccgagtgattgcagcaaggtcacgaaggttgtctgagcgtagtacatatcgaggttgaagtaggaggtcagagcggccttgaatgtgtggtggacgtccacgaagtgacacttcttgcagttttgagcggcggtctcatcgttgcagacgtcctgtgagtgtgggatttcgatgccagtctccttaaccaggttgtagctgatcatgaagcggatcttatcgaaggtcacaacgaacacacggttgtcaaccatgtagtagttgtttgtgtactcgtagaccacgttagagacgtacttggcgaagatgatttcgaaaggcttcacctcggacttcttaacgacgaacatgtagtaaccggtttcagacatgtgatcggagaatctgttcgagttgtagtcgttatcgtcgaacctcatcaggtagggggcgaagtcgtttgtgaagtagtgagtgatctcctgggtggaagccactgtacagatgttagtgttgtggttgatggtttgttccagtgtagcgcatgactggatggtgctcttcttgtacttaggtctcaacttgatcttgttgaattgacccacaactccctgggagttatccaggtactcgtccaacttcctcttggtgcctgtggccgacggctggttgacaccagcagagtgttcgaaggactcggcgtggtaagctgagctaggagagggttgttcgaccactggctgttcgagtgactcgctgtagtaggcagaggacacagcttcctccaggttgtcagtggtcttgagcagacactccaccaaatcgttgtcagtgagcgagttaactgaggcgaggaagttgctagcggcagcggtttcagagtcggagatgacagtatcagctccgtccggggttgggtggttgtagtaagacaagtaatcgttaggttgcttgtcgcagaactccgagtatgagttgtcgaagctagcacgagagggagtgctggcagaggtgtaggaagcgttgaagttgatttgagtcatggtgacctggttgttcacgatcttatcgccacctgtgtccacctgcagttgctgggcctcagcgcaggctgaagtggcctcacaggagtaggggctggaagcacagttggaagtcatgatgttttcttggacgttcaggacgtggctggatgtacggatcatgcgcccgatggtgggacggtatgaataatccggaatatttataggtttttttattacaaaactgttacgaaaacagtaaaatacttatttatttgcgagatggttatcattttaattatctccatgatcggatctcctaggctcaagcagtgatcagatccagacatgataagatacattgatgagtttggacaaaccacaactagaatgcagtgaaaaaaatgctttatttgtgaaatttgtgatgctattgctttatttgtaaccattataagctgcaataaacaagttaacaacaacaattgcatttgtctagtacttctcgacggtaccgcatgctatgcatcagctgctagcaccatggctcgagttacaggggacgggtgaggaaacgggtgccaatggggcgaggctcagtataaagtccattgttgtccacagtgaaatcaacgttggcagattttgcatagttagatgtatactgcacttcgggattccagcgtttgctgttttctttctgcagctcccattcaatctccacgctcacttgtcctgtggaatactgggtgatgaatgaagcaaactttgtagccgaaaactctgccggaggattcgcaggaacaggcgtgtttttgatgaggatctgaggaggcgggtgcttaagtccaaagccgcccatgagaggagacgggtgaaagtgtccatccgtgtgaggaattttggcccaaataggaccctgcaggtatacgtctctgtcttgccacaccattccaggtaaggctcccataacatgcacatctccggtcgcagggtctgtgctgctgctctggagattgactgccacagtcccaaatctttcggtggccacggggttagtggctttgatttcctcttcgtctgtgatcatgacattgtccaatgcagtgtttgaagctccggcgctctcctttccaaaaatcatgacaccgctcatgggaaagaacttgtctttgtcgtctttgtgtgaggccatagcagtgccagggttgattatagattcacgcccattaaggttatattttgaagcaccagtccaggtaaagttgctgttgttgttgtctgtttttgttttagaaacgcgctgctgccggtaacagggtccaggtagccagtttttgggctgaacagacatgccagctggagacccccggctaaacagcaagtccttgttttgggcacttccggactgattctgagttctgttcaggaaatacaggtactggtcgatgagaggattcatcagccggtccaggctctggctgtgcgcgtagctgctgtggaaaggcacgtcctcgaaggtgtagctgaaggtaaagttattgcccgttctcagcatctgcgatgggaaatattccaggcagtaaaaggatgaccgtcccactgcctggctgccattgttgagcgttaggtagccgtactgcggaatcatgaacacgtccgccgggaacggagggaggcagccctggtgcgcagagccgaggacgtacggcaactggtactccgagtccgagaagacttgaaccgtgctggtaaggttattagcgatggtcgtgacgccatcattcgtcgtgacctccttgacttggatgttgaagagcttgaagttgagtctcttgggccggaatccccaattgttgttgatgagtcgctgccagtcacgtggtgagaaatggcagtggaatctgttgaaatcaaaatacccccagggggtgctgtagccgaagtagtggttgtcgttgctggcccccgttgaagcactggagatttgcttgtagaggtggttgttataggtgggcaaggcccatgttcgggtgctggtggtgatgactctgtcgcccagccatgtggaatcgcaatgccaatttcctgaggcattacccactccgtcggcgccttcgttattgtctgccattggtgcgccaccgcctgaagccattgtagtaggtcccacagcagcgggggttgctggaggttctccgagaggttgtgggtcggggactgactctgagtcgccagtctgaccaaaattgagtctctttttagcgggctgctggcctgtcttgccaatgcccgaggaggagtctggctcttgtggcgactgctctaccggacgtttctttccaggagccgtcttagcaccttcctcaacgagaccaagaggttcgagaaccctcttcttggcctggaagactgctcgcccgaggttgcccccaaaagaggtatcttcttggagacgctcctgaaactcggcgtcggcgtggttataccggaggtacggattgtcacccgctttgagctgctggtcgtaggccttgtcgtgctcgagggccgctgcgtccgccgcgttgacgggctcccccttgtcgagtccgttgaagggtccgaggtacttgtagccaggaaggacgagaccccggccgtcgtcctgcttttgctggttggctttgggtttcggggctccaggtttgaggtcccaccactcgcggatgccctcagagaggttgtcctcgagccaatctggaagataaccgtcggcagccgtggcggctcaagtcttcgtcgagtgattgtaaataaaatgtaatttacagtatagtattttaattaatatacaaatgatttgataataattcttatttaactataatatattgtgttgggttgaattaaaggtccgtatctccagactgcagtttaaattgtgtaatttatgtagctgtaatttttaccttattaatattttttacgctttgcattcgacgactgaactcccaaatatatgtttaactcgtcttggtcgtttgaatttttgttgctgtgtttcctaatattttccatcaccttaaatatgttattgtaatcctcaatgttgaacttgcaattggacacggcatagttttccatagtcgtgtaaaacatggtattggctgcattgtaatacatccgactgagcgggtacggatctatgtgtttgagcagcctgttcaaaaactctgcatcgtcgcaaaacggaatttggtcacgatcccggtccgaagcgcgcggaattcaaagcgctacgtcagcgacgtcatcgattattgctccaatactagggttttgttttactatctgttctgcggtccacacatcttcttcgctagtcacgtacgcaaacaactcgggccgcaaaggtgttttaaaacatatcagattagaatcttttataacttggccgcattgtaaatagttgtgccaacgcgcgggaaacattttacacgtgctttcaatcttatctcataaacgcaactaaatatgatccttcaactcgctttacgagtagaattctacttgtaacgcacgattaattatgactcataagctgatgtcatgttttgcacacggctcataaccgaactcgctttacgagtagaattctacgcgtaaaacacaatcaagtatgagtcataagctgatgtcatgttttgcacacggctcataaccgaactggctttacgagtagaattctacttgtaacgcacgatcagtggatgatgtcataaacttatctcatgttttgcacacggctcataacttgagtcataagctgatatcagaagattattaacgtgtttaggtatgactcatttgttttcaaaactgaactcgctttacggatagaattctacttgtaaaacacaatcaggggatgatgtcattatacaaatgatgtcatttgtttttcaaaactaaactcgctttacgggtagaattctacttgtaaaacacaatcgagggataatgtcatttgttattctcaaatatgatgtcatttaaatttttattatgcaagaattgtatgttgctgtgtcatttatgaatgttttatcgacaacttgtttatttgtttcattgacttgttgttgttcgtgattatgattaattataaatcttttgttggggtcaacatcgatgtatacgccgctacagggcgcgtactatggttgctttgacgtatgcgggcggccgctctagagatcatggagataattaaaatgataaccatctcgcaaataaataagtattttactgttttcgtaacagttttgtaataaaaaaacctataaatattccggattattcataccgtcccaccatcgggcgcggatccgccgccctggcggggttttacgagattgtgattaaggtccccagcgaccttgacgagcatctgcccggcatttctgacagctttgtgaactgggtggccgagaaggagtgggagttgccgccagattctgacttggatctgaatctgattgagcaggcacccctgaccgtggccgagaagctgcagcgcgactttctgacggagtggcgccgtgtgagtaaggccccggaggcccttttctttgtgcaatttgagaagggagagagctacttccacttacacgtgctcgtggaaaccaccggggtgaaatccttagttttgggacgtttcctgagtcagattcgcgaaaaactgattcagagaatttaccgcgggatcgagccgactttgccaaactggttcgcggtcacaaagaccagaaacggcgccggaggcgggaacaaggtggtggacgagtgctacatccccaattacttgctccccaaaacccagcctgagctccagtgggcgtggactaatttagaacagtatttaagcgcctgtttgaatctcacggagcgtaaacggttggtggcgcagcatctgacgcacgtgtcgcagacgcaggagcagaacaaagagaatcagaatcccaattctgacgcgccggtgatcagatcaaaaacttcagccaggtacatggagctggtcgggtggctcgtggacaaggggattacctcggagaagcagtggatacaggaggaccaggcctcatacatctccttcaatgcggcctccaactcgcggtcccaaatcaaggctgccttggacaatgcgggaaagattatgagcctgactaaaaccgcccccgactacctggtgggccagcagcccgtggaggacatttccagcaatcggatttataaaattttggaactaaacgggtacgatccccaatatgcggcttccgtctttctgggatgggccacgaaaaagttcggcaagaggaacaccatctggctgtttgggcctgcaactaccgggaagaccaacatcgcggaggccatagcccacactgtgcccttctacgggtgcgtaaactggaccaatgagaactttcccttcaacgactgtgtggacaagatggtgatctggtgggaggaggggaagatgaccgccaaggtcgtggagtcggccaaagccattctcggaggaagcaaggtgcgcgtggaccagaaatgcaagtcctcggcccagatagacccgactcccgtgatcgtcacctccaacaccaacatgtgcgccgtgattgacgggaactcaacgaccttcgaacaccagcagccgttgcaagaccggatgttcaaatttgaactcacccgccgtctggatcatgactttgggaaggtcaccaagcaggaagtcaaagactttttccggtgggcaaaggatcacgtggttgaggtggagcatgaattctacgtcaaaaagggtggagccaagaaaagacccgcccccagtgacgcagatataagtgagcccaaacgggtgcgcgagtcagttgcgcagccatcgacgtcagacgcggaagcatcgatcaactacgcagacaggtaccaaaacaaatgttctcgtcacgtgggcatgaatctgatgctgtttccctgcagacaatgcgagagaatgaatcagaattcaaatatctgcttcactcacggacagaaagactgtttagagtgctttcccgtgtcagaatctcaacccgtttctgtcgtcaaaaaggcgtatcagaaactgtgctacattcatcatatcatgggaaaggtgccagacgcttgcactgcctgcgatctggtcaatgtggatttggatgactgcatctttgaacaataatctagagcctgcagtctcgacaagcttgtcgagaagtactagaggatcataatcagccataccacatttgtagaggttttacttgctttaaaaaacctcccacacctccccctgaacctgaaacataaaatgaatgcaattgttgttgttaacttgtttattgcagcttataatggttacaaataaagcaatagcatcacaaatttcacaaataaagcatttttttcactgcattctagttgtggtttgtccaaactcatcaatgtatcttatcatgtctggatctgatcactgcttgagcctaggagatccgaaccagataagtgaaatctagttccaaactattttgtcatttttaattttcgtattagcttacgacgctacacccagttcccatctattttgtcactcttccctaaataatccttaaaaactccatttccacccctcccagttcccaactattttgtccgcccacagcggggcatttttcttcctgttatgtttttaatcaaacatcctgccaactccatgtgacaaaccgtcatcttcggctactttttctctgtcacagaatgaaaatttttctgtcatctcttcgttattaatgtttgtaattgactgaatatcaacgcttatttgcagcctgaatggcgaatgggacgcgccctgtagcggcgcattaagcgcggcgggtgtggtggttacgcgcagcgtgaccgctacacttgccagcgccctagcgcccgctcctttcgctttcttcccttcctttctcgccacgttcgccggctttccccgtcaagctctaaatcgggggctccctttagggttccgatttagtgctttacggcacctcgaccccaaaaaacttgattagggtgatggttcacgtagtgggccatcgccctgatagacggtttttcgccctttgacgttggagtccacgttctttaatagtggactcttgttccaaactggaacaacactcaaccctatctcggtctattcttttgatttataagggattttgccgatttcggcctattggttaaaaaatgagctgatttaacaaaaatttaacgcgaattttaacaaaatattaacgtttacaatttcaggtggcacttttcggggaaatgtgcgcggaacccctatttgtttatttttctaaatacattcaaatatgtatccgctcatgagacaataaccctgataaatgcttcaataatattgaaaaaggaagagtatgagtattcaacatttccgtgtcgcccttattcccttttttgcggcattttgccttcctgtttttgctcacccagaaacgctggtgaaagtaaaagatgctgaagatcagttgggtgcacgagtgggttacatcgaactggatctcaacagcggtaagatccttgagagttttcgccccgaagaacgttttccaatgatgagcacttttaaagttctgctatgtggcgcggtattatcccgtattgacgccgggcaagagcaactcggtcgccgcatacactattctcagaatgacttggttgagtactcaccagtcacagaaaagcatcttacggatggcatgacagtaagagaattatgcagtgctgccataaccatgagtgataacactgcggccaacttacttctgacaacgatcggaggaccgaaggagctaaccgcttttttgcacaacatgggggatcatgtaactcgccttgatcgttgggaaccggagctgaatgaagccataccaaacgacgagcgtgacaccacgatgcctgtagcaatggcaacaacgttgcgcaaactattaactggcgaactacttactctagcttcccggcaacaattaatagactggatggaggcggataaagttgcaggaccacttctgcgctcggcccttccggctggctggtttattgctgataaatctggagccggtgagcgtgggtctcgcggtatcattgcagcactggggccagatggtaagccctcccgtatcgtagttatctacacgacggggagtcaggcaactatggatgaacgaaatagacagatcgctgagataggtgcctcactgattaagcattggtaactgtcagaccaagtttactcatatatactttagattgatttaaaacttcatttttaatttaaaaggatctaggtgaagatcctttttgataatctcatgaccaaaatcccttaacgtgagttttcgttccactgagcgtcagaccccgtagaaaagatcaaaggatcttcttgagatcctttttttctgcgcgtaatctgctgcttgcaaacaaaaaaaccaccgctaccagcggtggtttgtttgccggatcaagagctaccaactctttttccgaaggtaactggcttcagcagagcgcagataccaaatactgtccttctagtgtagccgtagttaggccaccacttcaagaactctgtagcaccgcctacatacctcgctctgctaatcctgttaccagtggctgctgccagtggcgataagtcgtgtcttaccgggttggactcaagacgatagttaccggataaggcgcagcggtcgggctgaacggggggttcgtgcacacagcccagcttggagcgaacgacctacaccgaactgagatacctacagcgtgagcattgagaaagcgccacgcttcccgaagggagaaaggcggacaggtatccggtaagcggcagggtcggaacaggagagcgcacgagggagcttccagggggaaacgcctggtatctttatagtcctgtcgggtttcgccacctctgacttgagcgtcgatttttgtgatgctcgtcaggggggcggagcctatggaaaaacgccagcaacgcggcctttttacggttcctggccttttgctggccttttgctcacatgttctttcctgcgttatcccctgattctgtggataaccgtattaccgcctttgagtgagctgataccgctcgccgcagccgaacgaccgagcgcagcgagtcagtgagcgaggaagcggaagagcgcctgatgcggtattttctccttacgcatctgtgcggtatttcacaccgcagaccagccgcgtaacctggcaaaatcggttacggttgagtaataaatggatgccctgcgtaagcgggtgtgggcggacaataaagtcttaaactgaacaaaatagatctaaactatgacaataaagtcttaaactagacagaatagttgtaaactgaaatcagtccagttatgctgtgaaaaagcatactggacttttgttatggctaaagcaaactcttcattttctgaagtgcaaattgcccgtcgtattaaagaggggcgtggccaagggcatggtaaagactatattcgcggcgttgtgacaatttaccgaacaactccgcggccgggaagccgatctcggcttgaacgaattgttaggtggcggtacttgggtcgatatcaaagtgcatcacttcttcccgtatgcccaactttgtatagagagccactgcgggatcgtcaccgtaatctgcttgcacgtagatcacataagcaccaagcgcgttggcctcatgcttgaggagattgatgagcgcggtggcaatgccctgcctccggtgctcgccggagactgcgagatcatagatatagatctcactacgcggctgctcaaacctgggcagaacgtaagccgcgagagcgccaacaaccgcttcttggtcgaaggcagcaagcgcgatgaatgtcttactacggagcaagttcccgaggtaatcggagtccggctgatgttgggagtaggtggctacgtctccgaactcacgaccgaaaagatcaagagcagcccgcatggatttgacttggtcagggccgagcctacatgtgcgaatgatgcccatacttgagccacctaactttgttttagggcgactgccctgctgcgtaacatcgttgctgctgcgtaacatcgttgctgctccataacatcaaacatcgacccacggcgtaacgcgcttgctgcttggatgcccgaggcatagactgtacaaaaaaacagtcataacaagccatgaaaaccgccactgcgccgttaccaccgctgcgttcggtcaaggttct

SEQ ID NO: 13 - DNA, 2211 bp, Adeno-associated virus 1
  source 1..2211: mol_type = genomic DNA
atggctgccgatggttatcttccagattggctcgaggacaacctctctgagggcattcgcgagtggtgggacttgaaacctggagccccgaagcccaaagccaaccagcaaaagcaggacgacggccggggtctggtgcttcctggctacaagtacctcggacccttcaacggactcgacaagggggagcccgtcaacgcggcggacgcagcggccctcgagcacgacaaggcctacgaccagcagctcaaagcgggtgacaatccgtacctgcggtataaccacgccgacgccgagtttcaggagcgtctgcaagaagatacgtcttttgggggcaacctcgggcgagcagtcttccaggccaagaagcgggttctcgaacctctcggtctggttgaggaaggcgctaagacggctcctggaaagaaacgtccggtagagcagtcgccacaagagccagactcctcctcgggcatcggcaagacaggccagcagcccgctaaaaagagactcaattttggtcagactggcgactcagagtcagtccccgatccacaacctctcggagaacctccagcaacccccgctgctgtgggacctactacaatggcttcaggcggtggcgcaccaatggcagacaataacgaaggcgccgacggagtgggtaatgcctcaggaaattggcattgcgattccacatggctgggcgacagagtcatcaccaccagcacccgcacctgggccttgcccacctacaataaccacctctacaagcaaatctccagtgcttcaacgggggccagcaacgacaaccactacttcggctacagcaccccctgggggtattttgatttcaacagattccactgccacttttcaccacgtgactggcagcgactcatcaacaacaattggggattccggcccaagagactcaacttcaaactcttcaacatccaagtcaaggaggtcacgacgaatgatggcgtcacaaccatcgctaataaccttaccagcacggttcaagtcttctcggactcggagtaccagcttccgtacgtcctcggctctgcgcaccagggctgcctccctccgttcccggcggacgtgttcatgattccgcaatacggctacctgacgctcaacaatggcagccaagccgtgggacgttcatccttttactgcctggaatatttcccttctcagatgctgagaacgggcaacaactttaccttcagctacacctttgaggaagtgcctttccacagcagctacgcgcacagccagagcctggaccggctgatgaatcctctcatcgaccaatacctgtattacctgaacagaactcaaaatcagtccggaagtgcccaaaacaaggacttgctgtttagccgtgggtctccagctggcatgtctgttcagcccaaaaactggctacctggaccctgttatcggcagcagcgcgtttctaaaacaaaaacagacaacaacaacagcaattttacctggactggtgcttcaaaatataacctcaatgggcgtgaatccatcatcaaccctggcactgctatggcctcacacaaagacgacgaagacaagttctttcccatgagcggtgtcatgatttttggaaaagagagcgccggagcttcaaacactgcattggacaatgtcatgattacagacgaagaggaaattaaagccactaaccctgtggccaccgaaagatttgggaccgtggcagtcaatttccagagcagcagcacagaccctgcgaccggagatgtgcatgctatgggagcattacctggcatggtgtggcaagatagagacgtgtacctgcagggtcccatttgggccaaaattcctcacacagatggacactttcacccgtctcctcttatgggcggctttggactcaagaacccgcctcctcagatcctcatcaaaaacacgcctgttcctgcgaatcctccggcggagttttcagctacaaagtttgcttcattcatcacccaatactccacaggacaagtgagtgtggaaattgaatgggagctgcagaaagaaaacagcaagcgctggaatcccgaagtgcagtacacatccaattatgcaaaatctgccaacgttgattttactgtggacaacaatggactttatactgagcctcgccccattggcacccgttaccttacccgtcccctgtaa

SEQ ID NO: 14 - DNA, 2208 bp, Adeno-associated virus 2
  source 1..2208: mol_type = genomic DNA
atggctgccgatggttatcttccagattggctcgaggacactctctctgaaggaataagacagtggtggaagctcaaacctggcccaccaccaccaaagcccgcagagcggcataaggacgacagcaggggtcttgtgcttcctgggtacaagtacctcggacccttcaacggactcgacaagggagagccggtcaacgaggcagacgccgcggccctcgagcacgacaaagcctacgaccggcagctcgacagcggagacaacccgtacctcaagtacaaccacgccgacgcggagtttcaggagcgccttaaagaagatacgtcttttgggggcaacctcggacgagcagtcttccaggcgaaaaagagggttcttgaacctctgggcctggttgaggaacctgttaagacggctccgggaaaaaagaggccggtagagcactctcctgtggagccagactcctcctcgggaaccggaaaggcgggccagcagcctgcaagaaaaagattgaattttggtcagactggagacgcagactcagtacctgacccccagcctctcggacagccaccagcagccccctctggtctgggaactaatacgatggctacaggcagtggcgcaccaatggcagacaataacgagggcgccgacggagtgggtaattcctcgggaaattggcattgcgattccacatggatgggcgacagagtcatcaccaccagcacccgaacctgggccctgcccacctacaacaaccacctctacaaacaaatttccagccaatcaggagcctcgaacgacaatcactactttggctacagcaccccttgggggtattttgacttcaacagattccactgccacttttcaccacgtgactggcaaagactcatcaacaacaactggggattccgacccaagagactcaacttcaagctctttaacattcaagtcaaagaggtcacgcagaatgacggtacgacgacgattgccaataaccttaccagcacggttcaggtgtttactgactcggagtaccagctcccgtacgtcctcggctcggcgcatcaaggatgcctcccgccgttcccagcagacgtcttcatggtgccacagtatggatacctcaccctgaacaacgggagtcaggcagtaggacgctcttcattttactgcctggagtactttccttctcagatgctgcgtaccggaaacaactttaccttcagctacacttttgaggacgttcctttccacagcagctacgctcacagccagagtctggaccgtctcatgaatcctctcatcgaccagtacctgtattacttgagcagaacaaacactccaagtggaaccaccacgcagtcaaggcttcagttttctcaggccggagcgagtgacattcgggaccagtctaggaactggcttcctggaccctgttaccgccagcagcgagtatcaaagacatctgcggataacaacaacagtgaatactcgtggactggagctaccaagtaccacctcaatggcagagactctctggtgaatccgggcccggccatggcaagccacaaggacgatgaagaaaagttttttcctcagagcggggttctcatctttgggaagcaaggctcagagaaaacaaatgtggacattgaaaaggtcatgattacagacgaagaggaaatcaggacaaccaatcccgtggctacggagcagtatggttctgtatctaccaacctccagagaggcaacagacaagcagctaccgcagatgtcaacacacaaggcgttcttccaggcatggtctggcaggacagagatgtgtaccttcaggggcccatctgggcaaagattccacacacggacggacattttcacccctctcccctcatgggtggattcggacttaaacaccctcctccacagattctcatcaagaacaccccggtacctgcgaatccttcgaccaccttcagtgcggcaaagtttgcttccttcatcacacagtactccacgggacaggtcagcgtggagatcgagtgggagctgcagaaggaaaacagcaaacgctggaatcccgaaattcagtacacttccaactacaacaagtctgttaatgtggactttactgtggacactaatggcgtgtattcagagcctcgccccattggcaccagatacctgactcgtaatctgtaa

SEQ ID NO: 15 - DNA, 2211 bp, Adeno-associated virus 3
  source 1..2211: mol_type = genomic DNA
atggctgctgacggttatcttccagattggctcgaggacaacctttctgaaggcattcgtgagtggtgggctctgaaacctggagtccctcaacccaaagcgaaccaacaacaccaggacaaccgtcggggtcttgtgcttccgggttacaaatacctcggacccggtaacggactcgacaaaggagagccggtcaacgaggcggacgcggcagccctcgaacacgacaaagcttacgaccagcagctcaaggccggtgacaacccgtacctcaagtacaaccacgccgacgccgagtttcaggagcgtcttcaagaagatacgtcttttgggggcaaccttggcagagcagtcttccaggccaaaaagaggatccttgagcctcttggtctggttgaggaagcagctaaaacggctcctggaaagaagaggcctgtagatcagtctcctcaggaaccggactcatcatctggtgttggcaaatcgggcaaacagcctgccagaaaaagactaaatttcggtcagactggcgactcagagtcagtcccagaccctcaacctctcggagaaccaccagcagcccccacaagtttgggatctaatacaatggcttcaggcggtggcgcaccaatggcagacaataacgagggtgccgatggagtgggtaattcctcaggaaattggcattgcgattcccaatggctgggcgacagagtcatcaccaccagcaccagaacctgggccctgcccacttacaacaaccatctctacaagcaaatctccagccaatcaggagcttcaaacgacaaccactactttggctacagcaccccttgggggtattttgactttaacagattccactgccacttctcaccacgtgactggcagcgactcattaacaacaactggggattccggcccaagaaactcagcttcaagctcttcaacatccaagttaaagaggtcacgcagaacgatggcacgacgactattgccaataaccttaccagcacggttcaagtgtttacggactcggagtatcagctcccgtacgtgctcgggtcggcgcaccaaggctgtctcccgccgtttccagcggacgtcttcatggtccctcagtatggatacctcaccctgaacaacggaagtcaagcggtgggacgctcatccttttactgcctggagtacttcccttcgcagatgctaaggactggaaataacttccaattcagctataccttcgaggatgtaccttttcacagcagctacgctcacagccagagtttggatcgcttgatgaatcctcttattgatcagtatctgtactacctgaacagaacgcaaggaacaacctctggaacaaccaaccaatcacggctgctttttagccaggctgggcctcagtctatgtctttgcaggccagaaattggctacctgggccctgctaccggcaacagagactttcaaagactgctaacgacaacaacaacagtaactttccttggacagcggccagcaaatatcatctcaatggccgcgactcgctggtgaatccaggaccagctatggccagtcacaaggacgatgaagaaaaatttttccctatgcacggcaatctaatatttggcaaagaagggacaacggcaagtaacgcagaattagataatgtaatgattacggatgaagaagagattcgtaccaccaatcctgtggcaacagagcagtatggaactgtggcaaataacttgcagagctcaaatacagctcccacgactagaactgtcaatgatcagggggccttacctggcatggtgtggcaagatcgtgacgtgtaccttcaaggacctatctgggcaaagattcctcacacggatggacactttcatccttctcctctgatgggaggctttggactgaaacatccgcctcctcaaatcatgatcaaaaatactccggtaccggcaaatcctccgacgactttcagcccggccaagtttgcttcatttatcactcagtactccactggacaggtcagcgtggaaattgagtgggagctacagaaagaaaacagcaaacgttggaatccagagattcagtacacttccaactacaacaagtctgttaatgtggactttactgtagacactaatggtgtttatagtgaacctcgccctattggaacccggtatctcacacgaaacttgtaa

SEQ ID NO: 16 - DNA, 2205 bp, Adeno-associated virus 4
  source 1..2205: mol_type = genomic DNA
atgactgacggttaccttccagattggctagaggacaacctctctgaaggcgttcgagagtggtgggcgctgcaacctggagcccctaaacccaaggcaaatcaacaacatcaggacaacgctcggggtcttgtgcttccgggttacaaatacctcggacccggcaacggactcgacaagggggaacccgtcaacgcagcggacgcggcagccctcgagcacgacaaggcctacgaccagcagctcaaggccggtgacaacccctacctcaagtacaaccacgccgacgcggagttccagcagcggcttcagggcgacacatcgtttgggggcaacctcggcagagcagtcttccaggccaaaaagagggttcttgaacctcttggtctggttgagcaagcgggtgagacggctcctggaaagaagagaccgttgattgaatccccccagcagcccgactcctccacgggtatcggcaaaaaaggcaagcagccggctaaaaagaagctcgttttcgaagacgaaactggagcaggcgacggaccccctgagggatcaacttccggagccatgtctgatgacagtgagatgcgtgcagcagctggcggagctgcagtcgagggcggacaaggtgccgatggagtgggtaatgcctcgggtgattggcattgcgattccacctggtctgagggccacgtcacgaccaccagcaccagaacctgggtcttgcccacctacaacaaccacctctacaagcgactcggagagagcctgcagtccaacacctacaacggattctccaccccctggggatactttgacttcaaccgcttccactgccacttctcaccacgtgactggcagcgactcatcaacaacaactggggcatgcgacccaaagccatgcgggtcaaaatcttcaacatccaggtcaaggaggtcacgacgtcgaacggcgagacaacggtggctaataaccttaccagcacggttcagatctttgcggactcgtcgtacgaactgccgtacgtgatggatgcgggtcaagagggcagcctgcctccttttcccaacgacgtctttatggtgccccagtacggctactgtggactggtgaccggcaacacttcgcagcaacagactgacagaaatgccttctactgcctggagtactttccttcgcagatgctgcggactggcaacaactttgaaattacgtacagttttgagaaggtgcctttccactcgatgtacgcgcacagccagagcctggaccggctgatgaaccctctcatcgaccagtacctgtggggactgcaatcgaccaccaccggaaccaccctgaatgccgggactgccaccaccaactttaccaagctgcggcctaccaacttttccaactttaaaaagaactggctgcccgggccttcaatcaagcagcagggcttctcaaagactgccaatcaaaactacaagatccctgccaccgggtcagacagtctcatcaaatacgagacgcacagcactctggacggaagatggagtgccctgacccccggacctccaatggccacggctggacctgcggacagcaagttcagcaacagccagctcatctttgcggggcctaaacagaacggcaacacggccaccgtacccgggactctgatcttcacctctgaggaggagctggcagccaccaacgccaccgatacggacatgtggggcaacctacctggcggtgaccagagcaacagcaacctgccgaccgtggacagactgacagccttgggagccgtgcctggaatggtctggcaaaacagagacatttactaccagggtcccatttgggccaagattcctcataccgatggacactttcacccctcaccgctgattggtgggtttgggctgaaacacccgcctcctcaaatttttatcaagaacaccccggtacctgcgaatcctgcaacgaccttcagctctactccggtaaactccttcattactcagtacagcactggccaggtgtcggtgcagattgactgggagatccagaaggagcggtccaaacgctggaaccccgaggtccagtttacctccaactacggacagcaaaactctctgttgtgggctcccgatgcggctgggaaatacactgagcctagggctatcggtacccgctacctcacccaccacctgtaa

SEQ ID NO: 17 - DNA, 2175 bp, Adeno-associated virus 5
  source 1..2175: mol_type = genomic DNA
atgtcttttgttgatcaccctccagattggttggaagaagttggtgaaggtcttcgcgagtttttgggccttgaagcgggcccaccgaaaccaaaacccaatcagcagcatcaagatcaagcccgtggtcttgtgctgcctggttataactatctcggacccggaaacggtctcgatcgaggagagcctgtcaacagggcagacgaggtcgcgcgagagcacgacatctcgtacaacgagcagcttgaggcgggagacaacccctacctcaagtacaaccacgcggacgccgagtttcaggagaagctcgccgacgacacatccttcgggggaaacctcggaaaggcagtctttcaggccaagaaaagggttctcgaaccttttggcctggttgaagagggtgctaagacggcccctaccggaaagcggatagacgaccactttccaaaaagaaagaaggctcggaccgaagaggactccaagccttccacctcgtcagacgccgaagctggacccagcggatcccagcagctgcaaatcccagcccaaccagcctcaagtttgggagctgatacaatgtctgcgggaggtggcggcccattgggcgacaataaccaaggtgccgatggagtgggcaatgcctcgggagattggcattgcgattccacgtggatgggggacagagtcgtcaccaagtccacccgaacctgggtgctgcccagctacaacaaccaccagtaccgagagatcaaaagcggctccgtcgacggaagcaacgccaacgcctactttggatacagcaccccctgggggtactttgactttaaccgcttccacagccactggagcccccgagactggcaaagactcatcaacaactactggggcttcagaccccggtccctcagagtcaaaatcttcaacattcaagtcaaagaggtcacggtgcaggactccaccaccaccatcgccaacaacctcacctccaccgtccaagtgtttacggacgacgactaccagctgccctacgtcgtcggcaacgggaccgagggatgcctgccggccttccctccgcaggtctttacgctgccgcagtacggttacgcgacgctgaaccgcgacaacacagaaaatcccaccgagaggagcagcttcttctgcctagagtactttcccagcaagatgctgagaacgggcaacaactttgagtttacctacaactttgaggaggtgcccttccactccagcttcgctcccagtcagaacctgttcaagctggccaacccgctggtggaccagtacttgtaccgcttcgtgagcacaaataacactggcggagtccagttcaacaagaacctggccgggagatacgccaacacctacaaaaactggttcccggggcccatgggccgaacccagggctggaacctgggctccggggtcaaccgcgccagtgtcagcgccttcgccacgaccaataggatggagctcgagggcgcgagttaccaggtgcccccgcagccgaacggcatgaccaacaacctccagggcagcaacacctatgccctggagaacactatgatcttcaacagccagccggcgaacccgggcaccaccgccacgtacctcgagggcaacatgctcatcaccagcgagagcgagacgcagccggtgaaccgcgtggcgtacaacgtcggcgggcagatggccaccaacaaccagagctccaccactgcccccgcgaccggcacgtacaacctccaggaaatcgtgcccggcagcgtgtggatggagagggacgtgtacctccaaggacccatctgggccaagatcccagagacgggggcgcactttcacccctctccggccatgggcggattcggactcaaacacccaccgcccatgatgctcatcaagaacacgcctgtgcccggaaatatcaccagcttctcggacgtgcccgtcagcagcttcatcacccagtacagcaccgggcaggtcaccgtggagatggagtgggagctcaagaaggaaaactccaagaggtggaacccagagatccagtacacaaacaactacaacgacccccagtttgtggactttgccccggacagcaccggggaatacagaaccaccagacctatcggaacccgataccttacccgacccctttaa

SEQ ID NO: 18 - DNA, 2211 bp, Adeno-associated virus 6
  source 1..2211: mol_type = genomic DNA
atggctgccgatggttatcttccagattggctcgaggacaacctctctgagggcattcgcgagtggtgggacttgaaacctggagccccgaaacccaaagccaaccagcaaaagcaggacgacggccggggtctggtgcttcctggctacaagtacctcggacccttcaacggactcgacaagggggagcccgtcaacgcggcggatgcagcggccctcgagcacgacaaggcctacgaccagcagctcaaagcgggtgacaatccgtacctgcggtataaccacgccgacgccgagtttcaggagcgtctgcaagaagatacgtcttttgggggcaacctcgggcgagcagtcttccaggccaagaagagggttctcgaacctcttggtctggttgaggaaggtgctaagacggctcctggaaagaaacgtccggtagagcagtcgccacaagagccagactcctcctcgggcattggcaagacaggccagcagcccgctaaaaagagactcaattttggtcagactggcgactcagagtcagtccccgacccacaacctctcggagaacctccagcaacccccgctgctgtgggacctactacaatggcttcaggcggtggcgcaccaatggcagacaataacgaaggcgccgacggagtgggtaatgcctcaggaaattggcattgcgattccacatggctgggcgacagagtcatcaccaccagcacccgaacatgggccttgcccacctataacaaccacctctacaagcaaatctccagtgcttcaacgggggccagcaacgacaaccactacttcggctacagcaccccctgggggtattttgatttcaacagattccactgccatttctcaccacgtgactggcagcgactcatcaacaacaattggggattccggcccaagagactcaacttcaagctcttcaacatccaagtcaaggaggtcacgacgaatgatggcgtcacgaccatcgctaataaccttaccagcacggttcaagtcttctcggactcggagtaccagttgccgtacgtcctcggctctgcgcaccagggctgcctccctccgttcccggcggacgtgttcatgattccgcagtacggctacctaacgctcaacaatggcagccaggcagtgggacggtcatccttttactgcctggaatatttcccatcgcagatgctgagaacgggcaataactttaccttcagctacaccttcgaggacgtgcctttccacagcagctacgcgcacagccagagcctggaccggctgatgaatcctctcatcgaccagtacctgtattacctgaacagaactcagaatcagtccggaagtgcccaaaacaaggacttgctgtttagccgggggtctccagctggcatgtctgttcagcccaaaaactggctacctggaccctgttaccggcagcagcgcgtttctaaaacaaaaacagacaacaacaacagcaactttacctggactggtgcttcaaaatataaccttaatgggcgtgaatctataatcaaccctggcactgctatggcctcacacaaagacgacaaagacaagttctttcccatgagcggtgtcatgatttttggaaaggagagcgccggagcttcaaacactgcattggacaatgtcatgatcacagacgaagaggaaatcaaagccactaaccccgtggccaccgaaagatttgggactgtggcagtcaatctccagagcagcagcacagaccctgcgaccggagatgtgcatgttatgggagccttacctggaatggtgtggcaagacagagacgtatacctgcagggtcctatttgggccaaaattcctcacacggatggacactttcacccgtctcctctcatgggcggctttggacttaagcacccgcctcctcagatcctcatcaaaaacacgcctgttcctgcgaatcctccggcagagttttcggctacaaagtttgcttcattcatcacccagtattccacaggacaagtgagcgtggagattgaatgggagctgcagaaagaaaacagcaaacgctggaatcccgaagtgcagtatacatctaactatgcaaaatctgccaacgttgatttcactgtggacaacaatggactttatactgagcctcgccccattggcacccgttacctcacccgtcccctgtaa

SEQ ID NO: 19 - DNA, 2214 bp, Adeno-associated virus 7
  source 1..2214: mol_type = genomic DNA
atggctgccgatggttatcttccagattggctcgaggacaacctctctgagggcattcgcgagtggtgggacctgaaacctggagccccgaaacccaaagccaaccagcaaaagcaggacaacggccggggtctggtgcttcctggctacaagtacctcggacccttcaacggactcgacaagggggagcccgtcaacgcggcggacgcagcggccctcgagcacgacaaggcctacgaccagcagctcaaagcgggtgacaatccgtacctgcggtataaccacgccgacgccgagtttcaggagcgtctgcaagaagatacgtcatttgggggcaacctcgggcgagcagtcttccaggccaagaagcgggttctcgaacctctcggtctggttgaggaaggcgctaagacggctcctgcaaagaagagaccggtagagccgtcacctcagcgttcccccgactcctccacgggcatcggcaagaaaggccagcagcccgccagaaagagactcaatttcggtcagactggcgactcagagtcagtccccgaccctcaacctctcggagaacctccagcagcgccctctagtgtgggatctggtacagtggctgcaggcggtggcgcaccaatggcagacaataacgaaggtgccgacggagtgggtaatgcctcaggaaattggcattgcgattccacatggctgggcgacagagtcattaccaccagcacccgaacctgggccctgcccacctacaacaaccacctctacaagcaaatctccagtgaaactgcaggtagtaccaacgacaacacctacttcggctacagcaccccctgggggtattttgactttaacagattccactgccacttctcaccacgtgactggcagcgactcatcaacaacaactggggattccggcccaagaagctgcggttcaagctcttcaacatccaggtcaaggaggtcacgacgaatgacggcgttacgaccatcgctaataaccttaccagcacgattcaggtattctcggactcggaataccagctgccgtacgtcctcggctctgcgcaccagggctgcctgcctccgttcccggcggacgtcttcatgattcctcagtacggctacctgactctcaacaatggcagtcagtctgtgggacgttcctccttctactgcctggagtacttcccctctcagatgctgagaacgggcaacaactttgagttcagctacagcttcgaggacgtgcctttccacagcagctacgcacacagccagagcctggaccggctgatgaatcccctcatcgaccagtacttgtactacctggccagaacacagagtaacccaggaggcacagctggcaatcgggaactgcagttttaccagggcgggccttcaactatggccgaacaagccaagaattggttacctggaccttgcttccggcaacaaagagtctccaaaacgctggatcaaaacaacaacagcaactttgcttggactggtgccaccaaatatcacctgaacggcagaaactcgttggttaatcccggcgtcgccatggcaactcacaaggacgacgaggaccgctttttcccatccagcggagtcctgatttttggaaaaactggagcaactaacaaaactacattggaaaatgtgttaatgacaaatgaagaagaaattcgtcctactaatcctgtagccacggaagaatacgggatagtcagcagcaacttacaagcggctaatactgcagcccagacacaagttgtcaacaaccagggagccttacctggcatggtctggcagaaccgggacgtgtacctgcagggtcccatctgggccaagattcctcacacggatggcaactttcacccgtctcctttgatgggcggctttggacttaaacatccgcctcctcagatcctgatcaagaacactcccgttcccgctaatcctccggaggtgtttactcctgccaagtttgcttcgttcatcacacagtacagcaccggacaagtcagcgtggaaatcgagtgggagctgcagaaggaaaacagcaagcgctggaacccggagattcagtacacctccaactttgaaaagcagactggtgtggactttgccgttgacagccagggtgtttactctgagcctcgccctattggcactcgttacctcacccgtaatctgtaa

SEQ ID NO: 20 - DNA, 2217 bp, Adeno-associated virus 8; identical to SEQ ID NO: 2
  source 1..2217: mol_type = genomic DNA

SEQ ID NO: 21 - DNA, 2211 bp, Adeno-associated virus 9
  source 1..2211: mol_type = genomic DNA
atggctgccgatggttatcttccagattggctcgaggacaaccttagtgaaggaattcgcgagtggtgggctttgaaacctggagcccctcaacccaaggcaaatcaacaacatcaagacaacgctcgaggtcttgtgcttccgggttacaaataccttggacccggcaacggactcgacaagggggagccggtcaacgcagcagacgcggcggccctcgagcacgacaaggcctacgaccagcagctcaaggccggagacaacccgtacctcaagtacaaccacgccgacgccgagttccaggagcggctcaaagaagatacgtcttttgggggcaacctcgggcgagcagtcttccaggccaaaaagaggcttcttgaacctcttggtctggttgaggaagcggctaagacggctcctggaaagaagaggcctgtagagcagtctcctcaggaaccggactcctccgcgggtattggcaaatcgggtgcacagcccgctaaaaagagactcaatttcggtcagactggcgacacagagtcagtcccagaccctcaaccaatcggagaacctcccgcagccccctcaggtgtgggatctcttacaatggcttcaggtggtggcgcaccagtggcagacaataacgaaggtgccgatggagtgggtagttcctcgggaaattggcattgcgattcccaatggctgggggacagagtcatcaccaccagcacccgaacctgggccctgcccacctacaacaatcacctctacaagcaaatctccaacagcacatctggaggatcttcaaatgacaacgcctacttcggctacagcaccccctgggggtattttgacttcaacagattccactgccacttctcaccacgtgactggcagcgactcatcaacaacaactggggattccggcctaagcgactcaacttcaagctcttcaacattcaggtcaaagaggttacggacaacaatggagtcaagaccatcgccaataaccttaccagcacggtccaggtcttcacggactcagactatcagctcccgtacgtgctcgggtcggctcacgagggctgcctcccgccgttcccagcggacgttttcatgattcctcagtacgggtatctgacgcttaatgatggaagccaggccgtgggtcgttcgtccttttactgcctggaatatttcccgtcgcaaatgctaagaacgggtaacaacttccagttcagctacgagtttgagaacgtacctttccatagcagctacgctcacagccaaagcctggaccgactaatgaatccactcatcgaccaatacttgtactatctctcaaagactattaacggttctggacagaatcaacaaacgctaaaattcagtgtggccggacccagcaacatggctgtccagggaagaaactacatacctggacccagctaccgacaacaacgtgtctcaaccactgtgactcaaaacaacaacagcgaatttgcttggcctggagcttcttcttgggctctcaatggacgtaatagcttgatgaatcctggacctgctatggccagccacaaagaaggagaggaccgtttctttcctttgtctggatctttaatttttggcaaacaaggaactggaagagacaacgtggatgcggacaaagtcatgataaccaacgaagaagaaattaaaactactaacccggtagcaacggagtcctatggacaagtggccacaaaccaccagagtgcccaagcacaggcgcagaccggctgggttcaaaaccaaggaatacttccgggtatggtttggcaggacagagatgtgtacctgcaaggacccatttgggccaaaattcctcacacggacggcaactttcacccttctccgctgatgggagggtttggaatgaagcacccgcctcctcagatcctcatcaaaaacacacctgtacctgcggatcctccaacggccttcaacaaggacaagctgaactctttcatcacccagtattctactggccaagtcagcgtggagatcgagtgggagctgcagaaggaaaacagcaagcgctggaacccggagatccagtacacttccaactattacaagtctaataatgttgaatttgctgttaatactgaaggtgtatatagtgaaccccgccccattggcaccagatacctgactcgtaatctgtaa

SEQ ID NO: 22 - DNA, 2211 bp, synthetic construct
  source 1..2211: mol_type = other DNA
acggctgccgatggttatcttccagattggctcgaggacaaccttagtgaaggaattcgcgagtggtgggctttgaaacctggagcccctcaacccaaggcaaatcaacaacatcaagacaacgctcgaggtcttgtgcttccgggttacaaataccttggacccggcaacggactcgacaagggggagccggtcaacgcagcagacgcggcggccctcgagcacgacaaggcctacgaccagcagctcaaggccggagacaacccgtacctcaagtacaaccacgccgacgccgagttccaggagcggctcaaagaagatacgtcttttgggggcaacctcgggcgagcagtcttccaggccaaaaagaggcttcttgaacctcttggtctggttgaggaagcggctaagacggctcctggaaagaagaggcctgtagagcagtctcctcaggaaccggactcctccgcgggtattggcaaatcgggtgcacagcccgctaaaaagagactcaatttcggtcagactggcgacacagagtcagtcccagaccctcaaccaatcggagaacctcccgcagccccctcaggtgtgggatctcttacaatggcttcaggtggtggcgcaccagtggcagacaataacgaaggtgccgatggagtgggtagttcctcgggaaattggcattgcgattcccaatggctgggggacagagtcatcaccaccagcacccgaacctgggccctgcccacctacaacaatcacctctacaagcaaatctccaacagcacatctggaggatcttcaaatgacaacgcctacttcggctacagcaccccctgggggtattttgacttcaacagattccactgccacttctcaccacgtgactggcagcgactcatcaacaacaactggggattccggcctaagcgactcaacttcaagctcttcaacattcaggtcaaagaggttacggacaacaatggagtcaagaccatcgccaataaccttaccagcacggtccaggtcttcacggactcagactatcagctcccgtacgtgctcgggtcggctcacgagggctgcctcccgccgttcccagcggacgttttcatgattcctcagtacgggtatctgacgcttaatgatggaagccaggccgtgggtcgttcgtccttttactgcctggaatatttcccgtcgcaaatgctaagaacgggtaacaacttccagttcagctacgagtttgagaacgtacctttccatagcagctacgctcacagccaaagcctggaccgactaatgaatccactcatcgaccaatacttgtactatctctcaaagactattaacggttctggacagaatcaacaaacgctaaaattcagtgtggccggacccagcaacatggctgtccagggaagaaactacatacctggacccagctaccgacaacaacgtgtctcaaccactgtgactcaaaacaacaacagcgaatttgcttggcctggagcttcttcttgggctctcaatggacgtaatagcttgatgaatcctggacctgctatggccagccacaaagaaggagaggaccgtttctttcctttgtctggatctttaatttttggcaaacaaggaactggaagagacaacgtggatgcggacaaagtcatgataaccaacgaagaagaaattaaaactactaacccggtagcaacggagtcctatggacaagtggccacaaaccaccagagtgcccaagcacaggcgcagaccggctgggttcaaaaccaaggaatacttccgggtatggtttggcaggacagagatgtgtacctgcaaggacccatttgggccaaaattcctcacacggacggcaactttcacccttctccgctgatgggagggtttggaatgaagcacccgcctcctcagatcctcatcaaaaacacacctgtacctgcggatcctccaacggccttcaacaaggacaagctgaactctttcatcacccagtattctactggccaagtcagcgtggagatcgagtgggagctgcagaaggaaaacagcaagcgctggaacccggagatccagtacacttccaactattacaagtctaataatgttgaatttgctgttaatactgaaggtgtatatagtgaaccccgccccattggcaccagatacctgactcgtaatctgtaa

SEQ ID NO: 23 - DNA, 411 bp, synthetic construct
  source 1..411: mol_type = other DNA
acggctgccgacggttatcttccagattggctcgaggacaaccttagcgaaggaatccgcgagtggtgggctttaaaacctggagcccctcaacccaaggcaaatcaacaacatcaagacaacgctcgaggtcttgtccttccgggttacaaataccttggacccggcaacggactcgacaagggggagccggtcaacgcagcagacgcggcggccctcgagcacgacaaggcctacgaccagcagctcaaggccggagacaacccgtacctcaagtacaaccacgccgacgccgagttccaggagcggctcaaagaagatacctcttttgggggcaacctcgggcgagcagtcttccaggccaaaaagaggcttcttgaacctcttggtctcgttgaggaagcggctaag

SEQ ID NO: 24 - DNA, 411 bp, synthetic construct
  source 1..411: mol_type = other DNA
acggctgccgacggttatcttccagattggctcgaggacaaccttagtgaaggaattcgcgagtggtgggctctaaaacctggagcccctcaacccaaggcaaatcaacaacatcaagacaacgctcgaggtcttgtccttccgggttacaaataccttggacccggcaacggactcgacaagggggagccggtcaacgcagcagacgcggcggccctcgagcacgacaaggcctacgaccagcagctcaaggccggagacaacccgtacctcaagtacaaccacgccgacgccgagttccaggagcggctcaaagaagatacctcttttgggggcaacctcgggcgagcagtcttccaggccaaaaagaggcttcttgaacctcttggtctcgttgaggaagcggctaag

SEQ ID NO: 25 - DNA, 411 bp, synthetic construct
  source 1..411: mol_type = other DNA
acggctgccgacggttatcttccagattggctcgaggacaaccttagtgaaggaattcgcgagtggtgggctctcaaacctggagcccctcaacccaaggcaaatcaacaacatcaagacaacgctcgaggtcttgtccttccgggttacaaataccttggacccggcaacggactcgacaagggggagccggtcaacgcagcagacgcggcggccctcgagcacgacaaggcctacgaccagcagctcaaggccggagacaacccgtacctcaagtacaaccacgccgacgccgagttccaggagcggctcaaagaagatacctcttttgggggcaacctcgggcgagcagtcttccaggccaaaaagaggcttcttgaacctcttggtctcgttgaggaagcggctaag

SEQ ID NO: 26 - DNA, 411 bp, synthetic construct
  source 1..411: mol_type = other DNA
acggctgccgacggttatcttccagattggctcgaggacaaccttagtgaaggaattcgcgagtggtgggctcttaaacctggagcccctcaacccaaggcaaatcaacaacatcaagacaacgctcgaggtcttgtccttccgggttacaaataccttggacccggcaacggactcgacaagggggagccggtcaacgcagcagacgcggcggccctcgagcacgacaaggcctacgaccagcagctcaaggccggagacaacccgtacctcaagtacaaccacgccgacgccgagttccaggagcggctcaaagaagatacctcttttgggggcaacctcgggcgagcagtcttccaggccaaaaagaggcttcttgaacctcttggtctcgttgaggaagcggctaag